European Patent Specification EP 3 594 335 B1, published May 1, 2024. Title: Carbohydrate Binding Module Variants and Polynucelotides Encoding Same. Applicant: Novozymes A/S Westh, Peter Borch, Kim Sorensen, Trine H Windahl, Michael S McBrayer, Brett. The sequence listing filed with the application follows.

SEQUENCE LISTING (100 sequences)

SEQ ID NO: 1 - DNA, 1893 bp, Trichoderma reesei
caactcagatcctccaggagacttgtacaccatcttttgaggcacagaaacccaatagtcaaccgcggactgcgcatcatgtatcggaagttggccgtcatctcggccttcttggccacagctcgtgctcagtcggcctgcactctccaatcggagactcacccgcctctgacatggcagaaatgctcgtctggtggcacgtgcactcaacagacaggctccgtggtcatcgacgccaactggcgctggactcacgctacgaacagcagcacgaactgctacgatggcaacacttggagctcgaccctatgtcctgacaacgagacctgcgcgaagaactgctgtctggacggtgccgcctacgcgtccacgtacggagttaccacgagcggtaacagcctctccattggctttgtcacccagtctgcgcagaagaacgttggcgctcgcctttaccttatggcgagcgacacgacctaccaggaattcaccctgcttggcaacgagttctctttcgatgttgatgtttcgcagctgccgtgcggcttgaacggagctctctacttcgtgtccatggacgcggatggtggcgtgagcaagtatcccaccaacaccgctggcgccaagtacggcacggggtactgtgacagccagtgtccccgcgatctgaagttcatcaatggccaggccaacgttgagggctgggagccgtcatccaacaacgcgaacacgggcattggaggacacggaagctgctgctctgagatggatatctgggaggccaactccatctccgaggctcttaccccccacccttgcacgactgtcggccaggagatctgcgagggtgatgggtgcggcggaacttactccgataacagatatggcggcacttgcgatcccgatggctgcgactggaacccataccgcctgggcaacaccagcttctacggccctggctcaagctttaccctcgataccaccaagaaattgaccgttgtcacccagttcgagacgtcgggtgccatcaaccgatactatgtccagaatggcgtcactttccagcagcccaacgccgagcttggtagttactctggcaacgagctcaacgatgattactgcacagctgaggaggcagaattcggcggatcctctttctcagacaagggcggcctgactcagttcaagaaggctacctctggcggcatggttctggtcatgagtctgtgggatgattactacgccaacatgctgtggctggactccacctacccgacaaacgagacctcctccacacccggtgccgtgcgcggaagctgctccaccagctccggtgtccctgctcaggtcgaatctcagtctcccaacgccaaggtcaccttctccaacatcaagttcggacccattggcagcaccggcaaccctagcggcggcaaccctcccggcggaaacccgcctggcaccaccaccacccgccgcccagccactaccactggaagctctcccggacctacccagtctcactacggccagtgcggcggtattggctacagcggccccacggtctgcgccagcggcacaacttgccaggtcctgaacccttactactctcagtgcctgtaaagctccgtggcgaaagcctgacgcaccggtagattcttggtgagcccgtatcatgacggcggcgggagctacatggccccgggtgatttattttttttgtatctacttctgacccttttcaaatatacggtcaactcatctttcactggagatgcggcctgcttggtattgcgatgttgtcagcttggcaaattgtggctttcgaaaacacaaaacgattccttagtagccatgcattttaagataacggaatagaagaaagaggaaatt

SEQ ID NO: 2 - protein, 514 aa, Trichoderma reesei
MYRKLAVISAFLATARAQSACTLQSETHPPLTWQKCSSGGTCTQQTGSVVIDANWRWTHATNSSTNCYDGNTWSSTLCPDNETCAKNCCLDGAAYASTYGVTTSGNSLSIGFVTQSAQKNVGARLYLMASDTTYQEFTLLGNEFSFDVDVSQLPCGLNGALYFVSMDADGGVSKYPTNTAGAKYGTGYCDSQCPRDLKFINGQANVEGWEPSSNNANTGIGGHGSCCSEMDIWEANSISEALTPHPCTTVGQEICEGDGCGGTYSDNRYGGTCDPDGCDWNPYRLGNTSFYGPGSSFTLDTTKKLTVVTQFETSGAINRYYVQNGVTFQQPNAELGSYSGNELNDDYCTAEEAEFGGSSFSDKGGLTQFKKATSGGMVLVMSLWDDYYANMLWLDSTYPTNETSSTPGAVRGSCSTSSGVPAQVESQSPNAKVTFSNIKFGPIGSTGNPSGGNPPGGNPPGTTTTRRPATTTGSSPGPTQSHYGQCGGIGYSGPTVCASGTTCQVLNPYYSQCL

SEQ ID NO: 3 - DNA, 108 bp, Trichoderma reesei
acccagtctcactacggccagtgcggcggtattggctacagcggccccacggtctgcgccagcggcacaacttgccaggtcctgaacccttactactctcagtgcctg

SEQ ID NO: 4 - protein, 36 aa, Trichoderma reesei
TQSHYGQCGGIGYSGPTVCASGTTCQVLNPYYSQCL

SEQ ID NO: 5 - DNA, 1638 bp, Humicola insolens
atgcgtaccgccaagttcgccaccctcgccgcccttgtggcctcggccgccgcccagcaggcgtgcagtctcaccaccgagaggcacccttccctctcttggaacaagtgcaccgccggcggccagtgccagaccgtccaggcttccatcactctcgactccaactggcgctggactcaccaggtgtctggctccaccaactgctacacgggcaacaagtgggatactagcatctgcactgatgccaagtcgtgcgctcagaactgctgcgtcgatggtgccgactacaccagcacctatggcatcaccaccaacggtgattccctgagcctcaagttcgtcaccaagggccagcactcgaccaacgtcggctcgcgtacctacctgatggacggcgaggacaagtatcagagtacgttctatcttcagccttctcgcgccttgaatcctggctaacgtttacacttcacagccttcgagctcctcggcaacgagttcaccttcgatgtcgatgtctccaacatcggctgcggtctcaacggcgccctgtacttcgtctccatggacgccgatggtggtctcagccgctatcctggcaacaaggctggtgccaagtacggtaccggctactgcgatgctcagtgcccccgtgacatcaagttcatcaacggcgaggccaacattgagggctggaccggctccaccaacgaccccaacgccggcgcgggccgctatggtacctgctgctctgagatggatatctgggaagccaacaacatggctactgccttcactcctcacccttgcaccatcattggccagagccgctgcgagggcgactcgtgcggtggcacctacagcaacgagcgctacgccggcgtctgcgaccccgatggctgcgacttcaactcgtaccgccagggcaacaagaccttctacggcaagggcatgaccgtcgacaccaccaagaagatcactgtcgtcacccagttcctcaaggatgccaacggcgatctcggcgagatcaagcgcttctacgtccaggatggcaagatcatccccaactccgagtccaccatccccggcgtcgagggcaattccatcacccaggactggtgcgaccgccagaaggttgcctttggcgacattgacgacttcaaccgcaagggcggcatgaagcagatgggcaaggccctcgccggccccatggtcctggtcatgtccatctgggatgaccacgcctccaacatgctctggctcgactcgaccttccctgtcgatgccgctggcaagcccggcgccgagcgcggtgcctgcccgaccacctcgggtgtccctgctgaggttgaggccgaggcccccaacagcaacgtcgtcttctccaacatccgcttcggccccatcggctcgaccgttgctggtctccccggcgcgggcaacggcggcaacaacggcggcaaccccccgccccccaccaccaccacctcctcggctccggccaccaccaccaccgccagcgctggccccaaggctggccgctggcagcagtgcggcggcatcggcttcactggcccgacccagtgcgaggagccctacatttgcaccaagctcaacgactggtactctcagtgcctgtaa

SEQ ID NO: 6 - protein, 525 aa, Humicola insolens
MRTAKFATLAALVASAAAQQACSLTTERHPSLSWNKCTAGGQCQTVQASITLDSNWRWTHQVSGSTNCYTGNKWDTSICTDAKSCAQNCCVDGADYTSTYGITTNGDSLSLKFVTKGQHSTNVGSRTYLMDGEDKYQTFELLGNEFTFDVDVSNIGCGLNGALYFVSMDADGGLSRYPGNKAGAKYGTGYCDAQCPRDIKFINGEANIEGWTGSTNDPNAGAGRYGTCCSEMDIWEANNMATAFTPHPCTIIGQSRCEGDSCGGTYSNERYAGVCDPDGCDFNSYRQGNKTFYGKGMTVDTTKKITVVTQFLKDANGDLGEIKRFYVQDGKIIPNSESTIPGVEGNSITQDWCDRQKVAFGDIDDFNRKGGMKQMGKALAGPMVLVMSIWDDHASNMLWLDSTFPVDAAGKPGAERGACPTTSGVPAEVEAEAPNSNVVFSNIRFGPIGSTVAGLPGAGNGGNNGGNPPPPTTTTSSAPATTTTASAGPKAGRWQQCGGIGFTGPTQCEEPYICTKLNDWYSQCL

SEQ ID NO: 7 - DNA, 110 bp, Humicola insolens
cccaaggctggccgctggcagcagtgcggcggcatcggcttcactggcccgacccagtgcgaggagccctacatttgcaccaagctcaacgactggtactctcagtgcct

SEQ ID NO: 8 - protein, 37 aa, Humicola insolens
PKAGRWQQCGGIGFTGPTQCEEPYICTKLNDWYSQCL

SEQ ID NO: 9 - DNA, 1593 bp, Chaetomium thermophilum
atgatgtacaagaagttcgccgctctcgccgccctcgtggctggcgccgccgcccagcaggcttgctccctcaccactgagacccaccccagactcacttggaagcgctgcacctctggcggcaactgctcgaccgtgaacggcgccgtcaccatcgatgccaactggcgctggactcacactgtttccggctcgaccaactgctacaccggcaacgagtgggatacctccatctgctctgatggcaagagctgcgcccagacctgctgcgtcgacggcgctgactactcttcgacctatggtatcaccaccagcggtgactccctgaacctcaagttcgtcaccaagcaccagcacggcaccaatgtcggctctcgtgtctacctgatggagaacgacaccaagtaccagatgttcgagctcctcggcaacgagttcaccttcgatgtcgatgtctctaacctgggctgcggtctcaacggcgccctctacttcgtctccatggacgctgatggtggtatgagcaagtactctggcaacaaggctggcgccaagtacggtaccggctactgcgatgctcagtgcccgcgcgaccttaagttcatcaacggcgaggccaacattgagaactggaccccttcgaccaatgatgccaacgccggtttcggccgctatggcagctgctgctctgagatggatatctgggatgccaacaacatggctactgccttcactcctcacccttgcaccattatcggccagagccgctgcgagggcaacagctgcggtggcacctacagctctgagcgctatgctggtgtttgcgatcctgatggctgcgacttcaacgcctaccgccagggcgacaagaccttctacggcaagggcatgaccgtcgacaccaccaagaagatgaccgtcgtcacccagttccacaagaactcggctggcgtcctcagcgagatcaagcgcttctacgttcaggacggcaagatcattgccaacgccgagtccaagatccccggcaaccccggcaactccatcacccaggagtggtgcgatgcccagaaggtcgccttcggtgacatcgatgacttcaaccgcaagggcggtatggctcagatgagcaaggccctcgagggccctatggtcctggtcatgtccgtctgggatgaccactacgccaacatgctctggctcgactcgacctaccccattgacaaggccggcacccccggcgccgagcgcggtgcttgcccgaccacctccggtgtccctgccgagattgaggcccaggtccccaacagcaacgttatcttctccaacatccgcttcggccccatcggctcgaccgtccctggcctcgacggcagcacccccagcaacccgaccgccaccgttgctcctcccacttctaccaccaccagcgtgagaagcagcactactcagatttccaccccgactagccagcccggcggctgcaccacccagaagtggggccagtgcggtggtatcggctacaccggctgcactaactgcgttgctggcactacctgcactgagctcaacccctggtacagccagtgcctgtaa

SEQ ID NO: 10 - protein, 530 aa, Chaetomium thermophilum
MMYKKFAALAALVAGAAAQQACSLTTETHPRLTWKRCTSGGNCSTVNGAVTIDANWRWTHTVSGSTNCYTGNEWDTSICSDGKSCAQTCCVDGADYSSTYGITTSGDSLNLKFVTKHQHGTNVGSRVYLMENDTKYQMFELLGNEFTFDVDVSNLGCGLNGALYFVSMDADGGMSKYSGNKAGAKYGTGYCDAQCPRDLKFINGEANIENWTPSTNDANAGFGRYGSCCSEMDIWDANNMATAFTPHPCTIIGQSRCEGNSCGGTYSSERYAGVCDPDGCDFNAYRQGDKTFYGKGMTVDTTKKMTVVTQFHKNSAGVLSEIKRFYVQDGKIIANAESKIPGNPGNSITQEWCDAQKVAFGDIDDFNRKGGMAQMSKALEGPMVLVMSVWDDHYANMLWLDSTYPIDKAGTPGAERGACPTTSGVPAEIEAQVPNSNVIFSNIRFGPIGSTVPGLDGSTPSNPTATVAPPTSTTTSVRSSTTQISTPTSQPGGCTTQKWGQCGGIGYTGCTNCVAGTTCTELNPWYSQCL

SEQ ID NO: 11 - DNA, 117 bp, Chaetomium thermophilum
ggcggctgcaccacccagaagtggggccagtgcggtggtatcggctacaccggctgcactaactgcgttgctggcactacctgcactgagctcaacccctggtacagccagtgcctg

SEQ ID NO: 12 - protein, 39 aa, Chaetomium thermophilum
GGCTTQKWGQCGGIGYTGCTNCVAGTTCTELNPWYSQCL

SEQ ID NO: 13 - DNA, 1614 bp, Talaromyces byssochlamydoides
atgtccgcctctctttcttacagactctacgaaaatgctctcattctctgttccctcgtggttgctgcccagggccagcagattggcaccttgcaggctgaggtccacccttctctgacttgggagacctgcagcaccggcggcagttgtaccaccatcgacggctctatcgtccttgatgccaactggcgctgggtccaccaggtcggcaccagcaccaactgctataccggcaatacctgggatacctccatctgcgataccgatacgacctgtgcccaagaatgcgctgtcgatggtgctgactacgagagcacctacggtatcaccaccagcggcaatgaagttcgtctcaactttgtcaccgacaactcgaatggagcgaacgtcggctcccgtgtctacctaatggcggatgacacccactaccagatcttcaatctgctgaaccaggagtttaccttcacagtggatgtctcaaacctgccctgcggtctcaacggcgccctctacctcgttgttatggatgccgacggtggtgtatccgagtatacgaataatgcggctggtgctcagtatggtgtgggctactgtgactcgcagtgtccccgagatctcaagttcatccaaggccaggccaacgttgagggctggacaccttcctccaataatgccaatactggtgttgggaacctcgggtcctgctgtgcagaaatagatatctgggaatcgaacagcatttctcaagcgcttaccgcccatccgtgcaacactcccacaaatacggtgtgtgatggcaacgcctgcggtggcacatacagcactactcgctatgctggcacttgtgatcctgatggctgtgatttcaacccgtaccggttgggcaacacgactttctatggtcctggcatgactattgataccacccagccgatcaccgttgtcactcagttcatcactgatgatggaacttccactggcaccttgtctgaaattaagcgctactacattcagaacgacgtcgtgtatgcccagcccaactccgacatcgctggcattactggaaatgtcattgatgccgcttactgtaccgctgagaattctgtcttccaagaagaaggttccttcgcacaacacggtggcatgagtggtgtcagtgaggctctgtccgctggtatggtcttggtcatgagcgtgtgggatgactacgacgccaatatgctgtggctcgacagcgactacccaaccaacgagtctacaagcacccccggtgtggcccgaggtagctgttccacttcctctggtgttcccgccaccgttgaatcccagagccctaactcctatgtgatctactcgaacatcaaggttggtcccatcggctcgaccttcagttccggtggttctggcagtggctctggcggcggttccggtggctctagcaccactacaaccaccacttcgtccacgcccacgactaccagctcttccggctctggcagtggcgtcgctcagcactggggacagtgcggtggtgagggctggactggcccaactacctgtgcctccccgtacacctgtcaggagcagaacccttactactcccagtgtctgtaa

SEQ ID NO: 14 - protein, 537 aa, Talaromyces byssochlamydoides
MSASLSYRLYENALILCSLVVAAQGQQIGTLQAEVHPSLTWETCSTGGSCTTIDGSIVLDANWRWVHQVGTSTNCYTGNTWDTSICDTDTTCAQECAVDGADYESTYGITTSGNEVRLNFVTDNSNGANVGSRVYLMADDTHYQIFNLLNQEFTFTVDVSNLPCGLNGALYLVVMDADGGVSEYTNNAAGAQYGVGYCDSQCPRDLKFIQGQANVEGWTPSSNNANTGVGNLGSCCAEIDIWESNSISQALTAHPCNTPTNTVCDGNACGGTYSTTRYAGTCDPDGCDFNPYRLGNTTFYGPGMTIDTTQPITVVTQFITDDGTSTGTLSEIKRYYIQNDVVYAQPNSDIAGITGNVIDAAYCTAENSVFQEEGSFAQHGGMSGVSEALSAGMVLVMSVWDDYDANMLWLDSDYPTNESTSTPGVARGSCSTSSGVPATVESQSPNSYVIYSNIKVGPIGSTFSSGGSGSGSGGGSGGSSTTTTTTSSTPTTTSSSGSGSGVAQHWGQCGGEGWTGPTTCASPYTCQEQNPYYSQCL

SEQ ID NO: 15 - DNA, 108 bp, Talaromyces byssochlamydoides
gtcgctcagcactggggacagtgcggtggtgagggctggactggcccaactacctgtgcctccccgtacacctgtcaggagcagaacccttactactcccagtgtctg

SEQ ID NO: 16 - protein, 36 aa, Talaromyces byssochlamydoides
VAQHWGQCGGEGWTGPTTCASPYTCQEQNPYYSQCL

SEQ ID NO: 17 - DNA, 1599 bp, Aspergillus fumigatus
atgctggcctccaccttctcctaccgcatgtacaagaccgcgctcatcctggccgcccttctgggctctggccaggctcagcaggtcggtacttcccaggcggaagtgcatccgtccatgacctggcagagctgcacggctggcggcagctgcaccaccaacaacggcaaggtggtcatcgacgcgaactggcgttgggtgcacaaagtcggcgactacaccaactgctacaccggcaacacctgggacacgactatctgccctgacgatgcgacctgcgcatccaactgcgcccttgagggtgccaactacgaatccacctatggtgtgaccgccagcggcaattccctccgcctcaacttcgtcaccaccagccagcagaagaacattggctcgcgtctgtacatgatgaaggacgactcgacctacgagatgtttaagctgctgaaccaggagttcaccttcgatgtcgatgtctccaacctcccctgcggtctcaacggtgctctgtactttgtcgccatggacgccggcggtggcatgtccaagtacccaaccaacaaggccggtgccaagtacggtactggatactgtgactcgcagtgccctcgcgacctcaagttcatcaacggtcaggccaacgttgaagggtggcagccctcctccaacgatgccaatgcgggtaccggcaaccacgggtcctgctgcgcggagatggatatctgggaggccaacagcatctccacggccttcaccccccatccgtgcgacacgcccggccaggtgatgtgcaccggtgatgcctgcggtggcacctacagctccgaccgctacggcggcacctgcgaccccgacggatgtgatttcaactccttccgccagggcaacaagaccttctacggccctggcatgaccgtcgacaccaagagcaagtttaccgtcgtcacccagttcatcaccgacgacggcacctccagcggcaccctcaaggagatcaagcgcttctacgtgcagaacggcaaggtgatccccaactcggagtcgacctggaccggcgtcagcggcaactccatcaccaccgagtactgcaccgcccagaagagcctgttccaggaccagaacgtcttcgaaaagcacggcggcctcgagggcatgggtgctgccctcgcccagggcatggttctcgtcatgtccctgtgggatgatcactcggccaacatgctctggctcgacagcaactacccgaccactgcctcttccaccactcccggcgtcgcccgtggtacctgcgacatctcctccggcgtccctgcggatgtcgaggcgaaccaccccgacgcctacgtcgtctactccaacatcaaggtcggccccatcggctcgaccttcaacagcggtggctcgaaccccggtggcggaaccaccacgacaactaccacccagcctactaccaccacgaccacggctggaaaccctggcggcaccggagtcgcacagcactatggccagtgtggtggaatcggatggaccggacccacaacctgtgccagcccttatacctgccagaagctgaatgattattactctcagtgcctgtag

SEQ ID NO: 18 - protein, 532 aa, Aspergillus fumigatus
MLASTFSYRMYKTALILAALLGSGQAQQVGTSQAEVHPSMTWQSCTAGGSCTTNNGKVVIDANWRWVHKVGDYTNCYTGNTWDTTICPDDATCASNCALEGANYESTYGVTASGNSLRLNFVTTSQQKNIGSRLYMMKDDSTYEMFKLLNQEFTFDVDVSNLPCGLNGALYFVAMDAGGGMSKYPTNKAGAKYGTGYCDSQCPRDLKFINGQANVEGWQPSSNDANAGTGNHGSCCAEMDIWEANSISTAFTPHPCDTPGQVMCTGDACGGTYSSDRYGGTCDPDGCDFNSFRQGNKTFYGPGMTVDTKSKFTVVTQFITDDGTSSGTLKEIKRFYVQNGKVIPNSESTWTGVSGNSITTEYCTAQKSLFQDQNVFEKHGGLEGMGAALAQGMVLVMSLWDDHSANMLWLDSNYPTTASSTTPGVARGTCDISSGVPADVEANHPDAYVVYSNIKVGPIGSTFNSGGSNPGGGTTTTTTTQPTTTTTTAGNPGGTGVAQHYGQCGGIGWTGPTTCASPYTCQKLNDYYSQCL

SEQ ID NO: 19 - DNA, 108 bp, Aspergillus fumigatus
gtcgcacagcactatggccagtgtggtggaatcggatggaccggacccacaacctgtgccagcccttatacctgccagaagctgaatgattattactctcagtgcctg

SEQ ID NO: 20 - protein, 36 aa, Aspergillus fumigatus
VAQHYGQCGGIGWTGPTTCASPYTCQKLNDYYSQCL

SEQ ID NO: 21 - DNA, 1581 bp, Thielavia terrestris
atgcacgccaagttcgcgaccctcgccgcccttgtggcgtccgccgcggcccagcaggcctgcacactcacggctgagaaccaccccaccctgtcgtggtccaagtgcacgtccggcggcagctgcaccagcgtctcgggctccgtcaccatcgatgccaactggcggtggactcaccaggtctcgagctcgaccaactgctacacgggcaatgagtgggacacgtccatctgcaccgacggtgcttcgtgcgccgccgcctgctgcctcgatggcgccgactactcgggcacctatggcatcaccaccagcggcaacgccctcagcctccagttcgtcactcagggcccctactcgaccaacattggctcgcgtacctacctgatggcctcggacaccaagtaccagatgttcactctgctcggcaacgagttcaccttcgacgtggacgtcacaggcctcggctgcggtctgaacggcgccctctacttcgtctccatggacgaggacggtggtctttccaagtactcgggcaacaaggctggcgccaagtacggcaccggctactgcgactcgcagtgcccccgcgacctcaagttcatcaacggcgaggctaacaacgttggctggaccccgtcgtccaacgacaagaacgccggcttgggcaactacggcagctgctgctccgagatggatgtctgggaggccaacagcatctcggcggcctacacgccccatccttgcactaccatcggccagacgcgctgcgagggcgacgactgcggtggtacctacagcactgaccgctacgccggcgagtgcgaccctgacggatgcgacttcaactcgtaccgcatgggcaacacgaccttctacggcaagggcatgaccgtcgacaccagcaagaagttcacggtggtgacccagttcctgacggactcgtctggcaacctgtccgagatcaagcgcttctacgtccagaacggcgtcgtcattcccaactcgaactccaacatcgcgggcgtctcgggcaactccatcacccaggccttctgcgatgctcagaagaccgctttcggcgacaccaacgtcttcgaccaaaagggcggcctggcccagatgggcaaggctcttgcccagcccatggtcctcgtcatgtccctctgggacgaccacgccgtcaacatgctctggctcgactcgacctacccgaccaacgcggccggcaagccgggcgccgcccgcggtacctgccccaccacctcgggcgtccccgccgacgtcgagtcccaggcgcccaactccaaggtcatctactccaacatccgcttcggccccatcggctccaccgtctccggcctgcccggcggcggcagcaaccccggcggcggctccagctccaccaccaccaccaccagacccgccacctccaccacctcctcggccagctccggcccgaccggcggtggcacggctgcccactggggccagtgcggcggcatcggctggaccggcccgaccgtctgcgcctcgccctacacctgccagaagctgaacgactggtactaccagtgcctctaa

SEQ ID NO: 22 - protein, 526 aa, Thielavia terrestris
MHAKFATLAALVASAAAQQACTLTAENHPTLSWSKCTSGGSCTSVSGSVTIDANWRWTHQVSSSTNCYTGNEWDTSICTDGASCAAACCLDGADYSGTYGITTSGNALSLQFVTQGPYSTNIGSRTYLMASDTKYQMFTLLGNEFTFDVDVTGLGCGLNGALYFVSMDEDGGLSKYSGNKAGAKYGTGYCDSQCPRDLKFINGEANNVGWTPSSNDKNAGLGNYGSCCSEMDVWEANSISAAYTPHPCTTIGQTRCEGDDCGGTYSTDRYAGECDPDGCDFNSYRMGNTTFYGKGMTVDTSKKFTVVTQFLTDSSGNLSEIKRFYVQNGVVIPNSNSNIAGVSGNSITQAFCDAQKTAFGDTNVFDQKGGLAQMGKALAQPMVLVMSLWDDHAVNMLWLDSTYPTNAAGKPGAARGTCPTTSGVPADVESQAPNSKVIYSNIRFGPIGSTVSGLPGGGSNPGGGSSSTTTTTRPATSTTSSASSGPTGGGTAAHWGQCGGIGWTGPTVCASPYTCQKLNDWYYQCL

SEQ ID NO: 23 - DNA, 108 bp, Thielavia terrestris
acggctgcccactggggccagtgcggcggcatcggctggaccggcccgaccgtctgcgcctcgccctacacctgccagaagctgaacgactggtactaccagtgcctc

SEQ ID NO: 24 - protein, 36 aa, Thielavia terrestris
TAAHWGQCGGIGWTGPTVCASPYTCQKLNDWYYQCL

SEQ ID NO: 25 - DNA, 1578 bp, Myceliophthora thermophilum
  misc_feature (1092)..(1092): n is a, c, g, or t
atgtacgccaagttcgcgaccctcgccgcccttgtggctggcgccgctgctcagaacgcctgcactctgaccgctgagaaccacccctcgctgacgtggtccaagtgcacgtctggcggcagctgcaccagcgtccagggttccatcaccatcgacgccaactggcggtggactcaccggaccgatagcgccaccaactgctacgagggcaacaagtgggatacttcgtactgcagcgatggtccttcttgcgcctccaagtgctgcatcgacggcgctgactactcgagcacctatggcatcaccacgagcggtaactccctgaacctcaagttcgtcaccaagggccagtactcgaccaacatcggctcgcgtacctacctgatggagagcgacaccaagtaccagttccagctcctcggcaacgagttcaccttcgatgtcgacgtctccaacctcggctgcggcctcaatggcgccctctacttcgtgtccatggatgccgatggtggcatgtccaagtactcgggcaacaaggcaggtgccaagtacggtaccggctactgtgattctcagtgcccccgcgacctcaagttcatcaacggcgaggccaacgtagagaactggcagagctcgaccaacgatgccaacgccggcacgggcaagtacggcagctgctgctccgagatggacgtctgggaggccaacaacatggccgccgccttcactccccacccttgcaccgtgatcggccagtcgcgctgcgagggcgactcgtgcggcggtacctacagcaccgaccgctatgccggcatctgcgaccccgacggatgcgacttcaactcgtaccgccagggcaacaagaccttctacggcaagggcatgacggtcgacacgaccaagaagatcacggtcgtcacccagttcctcaagaactcggccggcgagctctccgagatcaagcggttctacgtccagaacggcaaggtcatccccaactccgagtccaccatcccgggcgtcgagggcaactccatcacccaggactggtgcgaccgccagaaggccgccttcggcgacgtgaccgacttncaggacaagggcggcatggtccagatgggcaaggccctcgcggggcccatggtcctcgtcatgtccatctgggacgaccacgccgtcaacatgctctggctcgactccacctggcccatcgacggcgccggcaagccgggcgccgagcgcggtgcctgccccaccacctcgggcgtccccgctgaggtcgaggccgaggcccccaactccaacgtcatcttctccaacatccgcttcggccccatcggctccaccgtctccggcctgcccgacggcggcagcggcaaccccaacccgcccgtcagctcgtccaccccggtcccctcctcgtccaccacatcctccggttcctccggcccgactggcggcacgggtgtcgctaagcactatgagcaatgcggaggaatcgggttcactggccctacccagtgcgagagcccctacacttgcaccaagctgaatgactggtactcgcagtgcctgtaa

SEQ ID NO: 26 - protein, 525 aa, Myceliophthora thermophilum
  MISC_FEATURE (364)..(364): XAA = ANY AMINO ACID
MYAKFATLAALVAGAAAQNACTLTAENHPSLTWSKCTSGGSCTSVQGSITIDANWRWTHRTDSATNCYEGNKWDTSYCSDGPSCASKCCIDGADYSSTYGITTSGNSLNLKFVTKGQYSTNIGSRTYLMESDTKYQFQLLGNEFTFDVDVSNLGCGLNGALYFVSMDADGGMSKYSGNKAGAKYGTGYCDSQCPRDLKFINGEANVENWQSSTNDANAGTGKYGSCCSEMDVWEANNMAAAFTPHPCTVIGQSRCEGDSCGGTYSTDRYAGICDPDGCDFNSYRQGNKTFYGKGMTVDTTKKITVVTQFLKNSAGELSEIKRFYVQNGKVIPNSESTIPGVEGNSITQDWCDRQKAAFGDVTDXQDKGGMVQMGKALAGPMVLVMSIWDDHAVNMLWLDSTWPIDGAGKPGAERGACPTTSGVPAEVEAEAPNSNVIFSNIRFGPIGSTVSGLPDGGSGNPNPPVSSSTPVPSSSTTSSGSSGPTGGTGVAKHYEQCGGIGFTGPTQCESPYTCTKLNDWYSQCL

SEQ ID NO: 27 - DNA, 111 bp, Myceliophthora thermophilum
gtcgctaagcactatgagcaatgcggaggaatcgggttcactggccctacccagtgcgagagcccctacacttgcaccaagctgaatgactggtactcgcagtgcctgtaa

SEQ ID NO: 28 - protein, 36 aa, Myceliophthora thermophilum
VAKHYEQCGGIGFTGPTQCESPYTCTKLNDWYSQCL

SEQ ID NO: 29 - DNA, 1676 bp, Trichoderma reesei
  exon (1)..(461)
  sig_peptide (1)..(17)
  CDS (1)..(461)
  mat_peptide (52)..(1673)
  Intron (462)..(529)
  exon (530)..(1226)
  CDS (530)..(1226)
  Intron (1227)..(1289)
  exon (1290)..(1673)
  CDS (1290)..(1673)
atgtatcggaagttggccgtcatctcggccttcttggccacagctcgtgctcagtcggcctgcactctccaatcggagactcacccgcctctgacatggcagaaatgctcgtctggtggcacgtgcactcaacagacaggctccgtggtcatcgacgccaactggcgctggactcacgctacgaacagcagcacgaactgctacgatggcaacacttggagctcgaccctatgtcctgacaacgagacctgcgcgaagaactgctgtctggacggtgccgcctacgcgtccacgtacggagttaccacgagcggtaacagcctctccattggctttgtcacccagtctgcgcagaagaacgttggcgctcgcctttaccttatggcgagcgacacgacctaccaggaattcaccctgcttggcaacgagttctctttcgatgttgatgtttcgcagctgccgtaagtgacttaccatgaacccctgacgctatcttcttgttggctcccagctgactggccaattcaaggtgcggcttgaacggagctctctacttcgtgtccatggacgcggatggtggcgtgagcaagtatcccaccaacaccgctggcgccaagtacggcacggggtactgtgacagccagtgtccccgcgatctgaagttcatcaatggccaggccaacgttgagggctgggagccgtcatccaacaacgcgaacacgggcattggaggacacggaagctgctgctctgagatggatatctgggaggccaactccatctccgaggctcttaccccccacccttgcacgactgtcggccaggagatctgcgagggtgatgggtgcggcggaacttactccgataacagatatggcggcacttgcgatcccgatggctgcgactggaacccataccgcctgggcaacaccagcttctacggccctggctcaagctttaccctcgataccaccaagaaattgaccgttgtcacccagttcgagacgtcgggtgccatcaaccgatactatgtccagaatggcgtcactttccagcagcccaacgccgagcttggtagttactctggcaacgagctcaacgatgattactgcacagctgaggaggcagaattcggcggatcctctttctcagacaagggcggcctgactcagttcaagaaggctacctctggcggcatggttctggtcatgagtctgtgggatgatgtgagtttgatggacaaacatgcgcgttgacaaagagtcaagcagctgactgagatgttacagtactacgccaacatgctgtggctggactccacctacccgacaaacgagacctcctccacacccggtgccgtgcgcggaagctgctccaccagctccggtgtccctgctcaggtcgaatctcagtctcccaacgccaaggtcaccttctccaacatcaagttcggacccattggcagcaccggcaaccctagcggcggcaaccctcccggcggaaacccgcctggcaccaccaccacccgccgcccagccactaccactggaagctctcccggacctacccagtctcactacggccagtgcggcggtattggctacagcggccccacggtctgcgccagcggcacaacttgccaggtcctgaacccttactactctcagtgcctgtaa

SEQ ID NO: 30 - protein, 514 aa, Trichoderma reesei; identical to SEQ ID NO: 2

SEQ ID NO: 31 - DNA, 1545 bp, Trichoderma reesei
atgtatcggaagttggccgtcatctcggccttcttggccacagctcgtgctcagtcggcctgcactctccaatcggagactcacccgcctctgacatggcagaaatgctcgtctggtggcacgtgcactcaacagacaggctccgtggtcatcgacgccaactggcgctggactcacgctacgaacagcagcacgaactgctacgatggcaacacttggagctcgaccctatgtcctgacaacgagacctgcgcgaagaactgctgtctggacggtgccgcctacgcgtccacgtacggagttaccacgagcggtaacagcctctccattggctttgtcacccagtctgcgcagaagaacgttggcgctcgcctttaccttatggcgagcgacacgacctaccaggaattcaccctgcttggcaacgagttctctttcgatgttgatgtttcgcagctgccgtgcggcttgaacggagctctctacttcgtgtccatggacgcggatggtggcgtgagcaagtatcccaccaacaccgctggcgccaagtacggcacggggtactgtgacagccagtgtccccgcgatctgaagttcatcaatggccaggccaacgttgagggctgggagccgtcatccaacaacgcgaacacgggcattggaggacacggaagctgctgctctgagatggatatctgggaggccaactccatctccgaggctcttaccccccacccttgcacgactgtcggccaggagatctgcgagggtgatgggtgcggcggaacttactccgataacagatatggcggcacttgcgatcccgatggctgcgactggaacccataccgcctgggcaacaccagcttctacggccctggctcaagctttaccctcgataccaccaagaaattgaccgttgtcacccagttcgagacgtcgggtgccatcaaccgatactatgtccagaatggcgtcactttccagcagcccaacgccgagcttggtagttactctggcaacgagctcaacgatgattactgcacagctgaggaggcagaattcggcggatcctctttctcagacaagggcggcctgactcagttcaagaaggctacctctggcggcatggttctggtcatgagtctgtgggatgattactacgccaacatgctgtggctggactccacctacccgacaaacgagacctcctccacacccggtgccgtgcgcggaagctgctccaccagctccggtgtccctgctcaggtcgaatctcagtctcccaacgccaaggtcaccttctccaacatcaagttcggacccattggcagcaccggcaaccctagcggcggcaaccctcccggcggaaacccgcctggcaccaccaccacccgccgcccagccactaccactggaagctctcccggacctacccagtctcactacggccagtgcggcggtattggctacagcggccccacggtctgcgccagcggcacaacttgccaggtcctgaacccttactactctcagtgcctgtaa

SEQ ID NO: 32 - DNA, 1545 bp, Trichoderma reesei
atgtatcgtaagctcgcagtcatctccgcgttcctcgcaacagcacgagcgcagtccgcctgtaccttgcagtcggaaacacatcctcccctcacttggcagaaatgttcgtccggaggaacgtgtacgcagcagactggctcggtggtcatcgacgccaactggaggtggacgcatgcaaccaactcctccaccaactgttacgatggcaacacttggtcctccaccttgtgtcccgataacgaaacctgtgccaagaactgttgtttggatggtgcagcctacgcctcgacatacggagtcactacttccggcaactcgctctcgatcggcttcgtgactcagtccgcacagaaaaacgtcggagcgcgactctacttgatggcatccgatacaacctaccaggaattcactctcttgggcaacgagttctccttcgacgtcgacgtctcccagctcccttgtggcctcaacggagcactctacttcgtgtcgatggacgcggatggaggtgtctccaagtacccgaccaacacagcaggagcgaaatacggcacgggttactgtgactcgcagtgtcctcgcgatctcaagttcatcaacggccaggcaaacgtcgaaggctgggaaccctcgtcgaacaacgccaacaccggcattggaggccatggctcctgttgttcggaaatggatatctgggaggccaactcgatctccgaggcactcacaccccacccctgtacaaccgtcggccaggagatttgtgaaggagacggctgtggcggaacttactccgataaccgttacggtggtacctgtgatcccgatggctgtgactggaacccctaccgcctcggtaacacatcgttctacggtccgggttcctccttcaccctcgacactaccaaaaagttgacggtggtcacgcagttcgagacttccggagccatcaaccggtactacgtgcagaacggagtcacattccagcagcccaacgcagaactcggctcgtactcgggaaacgagctcaacgatgattactgtacagcggaagaggcagaattcggaggatcgtcgttctccgacaagggtggtttgacccagttcaagaaggccacatcgggaggaatggtgttggtcatgtccttgtgggacgactactatgccaacatgctctggctcgactccacctaccccaccaacgagacctcctcgacacctggcgcagtgaggggctcgtgttccacttcgtcgggagtgcctgcacaggtggagtcccagtcgccgaacgccaaggtcactttctccaacattaagttcggacccatcggttcgaccggcaacccctccggtggaaaccctcctggcggaaaccctcctggcacaactacaacacgacggcctgcgactacaacgggttcgtcccctggaccgacccagtcccactacggacagtgtggaggcatcggttattccggtccgaccgtctgtgcgtccggcacaacctgtcaggtcttgaacccttactattcgcagtgtctctaa

SEQ ID NO: 33 - DNA, 1545 bp, Trichoderma reesei
  sig_peptide (1)..(51)
  CDS (1)..(1542)
  mat_peptide (52)..(1542)
atgtatcgtaagctcgcagtcatctccgcgttcctcgcaacagcacgagcgcagtccgcctgtaccttgcagtcggaaacacatcctcccctcacttggcagaaatgttcgtccggaggaacgtgtacgcagcagactggctcggtggtcatcgacgccaactggaggtggacgcatgcaaccaactcctccaccaactgttacgatggcaacacttggtcctccaccttgtgtcccgataacgaaacctgtgccaagaactgttgtttggatggtgcagcctacgcctcgacatacggagtcactacttccggcaactcgctctcgatcggcttcgtgactcagtccgcacagaaaaacgtcggagcgcgactctacttgatggcatccgatacaacctaccaggaattcactctcttgggcaacgagttctccttcgacgtcgacgtctcccagctcccttgtggcctcaacggagcactctacttcgtgtcgatggacgcggatggaggtgtctccaagtacccgaccaacacagcaggagcgaaatacggcacgggttactgtgactcgcagtgtcctcgcgatctcaagttcatcaacggccaggcaaacgtcgaaggctgggaaccctcgtcggccaacgccgccaccggcattggaggccatggctcctgttgttcggaaatggatatctgggaggccaactcgatctccgaggcactcacaccccacccctgtacaaccgtcggccaggagatttgtgaaggagacggctgtggcggaacttactccgataaccgttacggtggtacctgtgatcccgatggctgtgactggaacccctaccgcctcggtaacacatcgttctacggtccgggttcctccttcaccctcgacactaccaaaaagttgacggtggtcacgcagttcgagacttccggagccatcaaccggtactacgtgcagaacggagtcacattccagcagcccaacgcagaactcggctcgtactcgggaaacgagctcaacgatgattactgtacagcggaagaggcagaattcggaggatcgtcgttctccgacaagggtggtttgacccagttcaagaaggccacatcgggaggaatggtgttggtcatgtccttgtgggacgactactatgccaacatgctctggctcgactccacctaccccaccaacgagacctcctcgacacctggcgcagtgaggggctcgtgttccacttcgtcgggagtgcctgcacaggtggagtcccagtcgccgaacgccaaggtcactttctccaacattaagttcggacccatcggttcgaccggcaacccctccggtggaaaccctcctggcggaaaccctcctggcacaactacaacacgacggcctgcgactacaacgggttcgtcccctggaccgacccagtcccactacggacagtgtggaggcatcggttattccggtccgaccgtctgtgcgtccggcacaacctgtcaggtcttgaacccttactattcgcagtgtctctaa

SEQ ID NO: 34 - protein, 514 aa, Trichoderma reesei
MYRKLAVISAFLATARAQSACTLQSETHPPLTWQKCSSGGTCTQQTGSVVIDANWRWTHATNSSTNCYDGNTWSSTLCPDNETCAKNCCLDGAAYASTYGVTTSGNSLSIGFVTQSAQKNVGARLYLMASDTTYQEFTLLGNEFSFDVDVSQLPCGLNGALYFVSMDADGGVSKYPTNTAGAKYGTGYCDSQCPRDLKFINGQANVEGWEPSSANAATGIGGHGSCCSEMDIWEANSISEALTPHPCTTVGQEICEGDGCGGTYSDNRYGGTCDPDGCDWNPYRLGNTSFYGPGSSFTLDTTKKLTVVTQFETSGAINRYYVQNGVTFQQPNAELGSYSGNELNDDYCTAEEAEFGGSSFSDKGGLTQFKKATSGGMVLVMSLWDDYYANMLWLDSTYPTNETSSTPGAVRGSCSTSSGVPAQVESQSPNAKVTFSNIKFGPIGSTGNPSGGNPPGGNPPGTTTTRRPATTTGSSPGPTQSHYGQCGGIGYSGPTVCASGTTCQVLNPYYSQCL

SEQ ID NO: 35 - DNA, 1599 bp, Aspergillus fumigatus
  sig_peptide (1)..(26)
  CDS (1)..(1596)
  mat_peptide (79)..(1596)
atgctggcctccaccttctcctaccgcatgtacaagaccgcgctcatcctggccgcccttctgggctctggccaggctcagcaggtcggtacttcccaggcggaagtgcatccgtccatgacctggcagagctgcacggctggcggcagctgcaccaccaacaacggcaaggtggtcatcgacgcgaactggcgttgggtgcacaaagtcggcgactacaccaactgctacaccggcaacacctgggacacgactatctgccctgacgatgcgacctgcgcatccaactgcgcccttgagggtgccaactacgaatccacctatggtgtgaccgccagcggcaattccctccgcctcaacttcgtcaccaccagccagcagaagaacattggctcgcgtctgtacatgatgaaggacgactcgacctacgagatgtttaagctgctgaaccaggagttcaccttcgatgtcgatgtctccaacctcccctgcggtctcaacggtgctctgtactttgtcgccatggacgccgacggtggcatgtccaagtacccaaccaacaaggccggtgccaagtacggtactggatactgtgactcgcagtgccctcgcgacctcaagttcatcaacggtcaggccaacgtcgaagggtggcagccctcctccaacgatgccaatgcgggtaccggcaaccacgggtcctgctgcgcggagatggatatctgggaggccaacagcatctccacggccttcaccccccatccgtgcgacacgcccggccaggtgatgtgcaccggtgatgcctgcggtggcacctacagctccgaccgctacggcggcacctgcgaccccgacggatgtgatttcaactccttccgccagggcaacaagaccttctacggccctggcatgaccgtcgacaccaagagcaagtttaccgtcgtcacccagttcatcaccgacgacggcacctccagcggcaccctcaaggagatcaagcgcttctacgtgcagaacggcaaggtgatccccaactcggagtcgacctggaccggcgtcagcggcaactccatcaccaccgagtactgcaccgcccagaagagcctgttccaggaccagaacgtcttcgaaaagcacggcggcctcgagggcatgggtgctgccctcgcccagggtatggttctcgtcatgtccctgtgggatgatcactcggccaacatgctctggctcgacagcaactacccgaccactgcctcttccaccactcccggcgtcgcccgtggtacctgcgacatctcctccggcgtccctgcggatgtcgaggcgaaccaccccgacgcctacgtcgtctactccaacatcaaggtcggccccatcggctcgaccttcaacagcggtggctcgaaccccggtggcggaaccaccacgacaactaccacccagcctactaccaccacgaccacggctggaaaccctggcggcaccggagtcgcacagcactatggccagtgtggtggaatcggatggaccggacccacaacctgtgccagcccttatacctgccagaagctgaatgattattactctcagtgcctgtag

SEQ ID NO: 36 - protein, 532 aa, Aspergillus fumigatus
MLASTFSYRMYKTALILAALLGSGQAQQVGTSQAEVHPSMTWQSCTAGGSCTTNNGKVVIDANWRWVHKVGDYTNCYTGNTWDTTICPDDATCASNCALEGANYESTYGVTASGNSLRLNFVTTSQQKNIGSRLYMMKDDSTYEMFKLLNQEFTFDVDVSNLPCGLNGALYFVAMDADGGMSKYPTNKAGAKYGTGYCDSQCPRDLKFINGQANVEGWQPSSNDANAGTGNHGSCCAEMDIWEANSISTAFTPHPCDTPGQVMCTGDACGGTYSSDRYGGTCDPDGCDFNSFRQGNKTFYGPGMTVDTKSKFTVVTQFITDDGTSSGTLKEIKRFYVQNGKVIPNSESTWTGVSGNSITTEYCTAQKSLFQDQNVFEKHGGLEGMGAALAQGMVLVMSLWDDHSANMLWLDSNYPTTASSTTPGVARGTCDISSGVPADVEANHPDAYVVYSNIKVGPIGSTFNSGGSNPGGGTTTTTTTQPTTTTTTAGNPGGTGVAQHYGQCGGIGWTGPTTCASPYTCQKLNDYYSQCL

SEQ ID NO: 37 - DNA, 1374 bp, Thermoascus aurantiacus
  sig_peptide (1)..(17)
  CDS (1)..(1371)
  mat_peptide (52)..(1371)
atgtatcagcgcgctcttctcttctctttcttcctctccgccgcccgcgcgcagcaggccggtaccctaaccgcagagaatcacccttccctgacctggcagcaatgctccagcggcggtagttgtaccacgcagaatggaaaagtcgttatcgatgcgaactggcgttgggtccataccacctctggatacaccaactgctacacgggcaatacgtgggacaccagtatctgtcccgacgacgtgacctgcgctcagaattgtgccttggatggagcggattacagtggcacctatggtgttacgaccagtggcaacgccctgagactgaactttgtcacccaaagctcagggaagaacattggctcgcgcctgtacctgctgcaggacgacaccacttatcagatcttcaagctgctgggtcaggagtttaccttcgatgtcgacgtctccaatctcccttgcgggctgaacggcgccctctactttgtggccatggacgccgacggcggattgtccaaataccctggcaacaaggcaggcgctaagtatggcactggttactgcgactctcagtgccctcgggatctcaagttcatcaacggtcaggccaacgttgaaggctggcagccgtctgccaacgacccaaatgccggcgttggtaaccacggttcctgctgcgctgagatggatgtctgggaagccaacagcatctctactgcggtgacgcctcacccatgcgacacccccggccagaccatgtgccagggagacgactgtggtggaacctactcctccactcgatatgctggtacctgcgaccctgatggctgcgacttcaatccttaccgccagggcaaccactcgttctacggccccgggaagatcgtcgacactagctccaaattcaccgtcgtcacccagttcatcaccgacgacgggaccccctccggcaccctgacggagatcaaacgcttctacgtccagaacggcaaggtgatcccccagtcggagtcgacgatcagcggcgtcaccggcaactcaatcaccaccgagtattgcacggcccagaaggccgccttcggcgacaacaccggcttcttcacgcacggcgggcttcagaagatcagtcaggctctggctcagggcatggtcctcgtcatgagcctgtgggacgatcacgccgccaacatgctctggctggacagcacctacccgactgatgcggacccggacacccctggcgtcgcgcgcggtacctgccccacgacctccggcgtcccggccgacgttgagtcgcagaaccccaattcatatgttatctactccaacatcaaggtcggacccatcaactcgaccttcaccgccaactaa

SEQ ID NO: 38 - protein, 457 aa, Thermoascus aurantiacus
MYQRALLFSFFLSAARAQQAGTLTAENHPSLTWQQCSSGGSCTTQNGKVVIDANWRWVHTTSGYTNCYTGNTWDTSICPDDVTCAQNCALDGADYSGTYGVTTSGNALRLNFVTQSSGKNIGSRLYLLQDDTTYQIFKLLGQEFTFDVDVSNLPCGLNGALYFVAMDADGGLSKYPGNKAGAKYGTGYCDSQCPRDLKFINGQANVEGWQPSANDPNAGVGNHGSCCAEMDVWEANSISTAVTPHPCDTPGQTMCQGDDCGGTYSSTRYAGTCDPDGCDFNPYRQGNHSFYGPGKIVDTSSKFTVVTQFITDDGTPSGTLTEIKRFYVQNGKVIPQSESTISGVTGNSITTEYCTAQKAAFGDNTGFFTHGGLQKISQALAQGMVLVMSLWDDHAANMLWLDSTYPTDADPDTPGVARGTCPTTSGVPADVESQNPNSYVIYSNIKVGPINSTFTAN

SEQ ID NO: 39 - DNA, 1428 bp, Penicillium emersonii
  exon (1)..(603)
  CDS (1)..(603)
  sig_peptide (1)..(18)
  mat_peptide (55)..(1425)
  Intron (604)..(663)
  exon (664)..(1425)
  CDS (664)..(1425)
atgcttcgacgggctcttcttctatcctcttccgccatccttgctgtcaaggcacagcaggccggcacggcgacggcagagaaccacccgcccctgacatggcaggaatgcaccgcccctgggagctgcaccacccagaacggggcggtcgttcttgatgcgaactggcgttgggtgcacgatgtgaacggatacaccaactgctacacgggcaatacctggaaccccacgtactgccctgacgacgaaacctgcgcccagaactgtgcgctggacggcgcggattacgagggcacctacggcgtgacttcgtcgggcagctccttgaagctcaatttcgtcaccgggtcgaacgtcggatcccgtctctacctgctgcaggacgactcgacctatcagatcttcaagcttctgaaccgcgagtttacctttgacgtcgatgtctccaatcttccgtgcggattgaacggcgctctgtactttgtcgccatggacgccgacggcggcgtgtccaagtacccgaacaacaaggctggtgccaagtacggaaccgggtattgcgactcccaatgcccacgggacctcaagttcatcgacggcgaggtatgtccagtggtaaaatcgatcgtctcgtgaacttctgctgacaggttcgatctacaggccaacgtcgagggctggcagccgtcttcgaacaacgccaacaccggaattggcgaccatggctcctgctgtgcggagatggatgtctgggaagccaacagcatctccaatgcggtcactccgcacccgtgcgacacgccaggccagacgatgtgctctggcgatgactgcggtggcacatactctaacgatcgctacgcgggaacctgcgatcctgacggctgtgacttcaacccttaccgcatgggcaacacttctttctacgggcctggcaagatcatcgataccaccaagcctttcactgtcgtgacgcagttcctcactgatgatggtacggatactggaactctcagcgagatcaagcgcttctacgtccagaacggcaacgtcattccgcagcccaactcggacatcagtggcgtgaccggcaactcgatcacgacggagttctgtactgctcagaagcaggcctttggcgacacggacgacttctctcagcacggtggcctggccaagatgggagcggccatgcagcagggtatggtcctggtgatgagtttgtgggacgactacgccgcgcagatgctgtggctggattccgactacccgacggatgcggaccccacgacccctggtattgcccgtggaacgtgtccgacggactcgggcgtcccatcggatgtcgagtcgcagagccccaactcctacgtgacctactcgaacatcaagtttggtccgatcaactcgaccttcaccgcttcgtga

SEQ ID NO: 40 - protein, 455 aa, Penicillium emersonii
MLRRALLLSSSAILAVKAQQAGTATAENHPPLTWQECTAPGSCTTQNGAVVLDANWRWVHDVNGYTNCYTGNTWNPTYCPDDETCAQNCALDGADYEGTYGVTSSGSSLKLNFVTGSNVGSRLYLLQDDSTYQIFKLLNREFTFDVDVSNLPCGLNGALYFVAMDADGGVSKYPNNKAGAKYGTGYCDSQCPRDLKFIDGEANVEGWQPSSNNANTGIGDHGSCCAEMDVWEANSISNAVTPHPCDTPGQTMCSGDDCGGTYSNDRYAGTCDPDGCDFNPYRMGNTSFYGPGKIIDTTKPFTVVTQFLTDDGTDTGTLSEIKRFYVQNGNVIPQPNSDISGVTGNSITTEFCTAQKQAFGDTDDFSQHGGLAKMGAAMQQGMVLVMSLWDDYAAQMLWLDSDYPTDADPTTPGIARGTCPTDSGVPSDVESQSPNSYVTYSNIKFGPINSTFTAS

SEQ ID NO: 41 - DNA, 1599 bp, Talaromyces leycettanus
  sig_peptide (1)..(25)
  CDS (1)..(1596)
  mat_peptide (76)..(1596)
atggccagcctcttctctttcaagatgtacaaggccgctctggtcctctcctctctccttgcggccacccaggcccagcaggccggcaccctgaccaccgaaacccatccttctctgacctggcagcaatgctctgccggcggcagctgcaccactcagaacggcaaggtcgtcatcgacgccaactggcgctgggttcacagcaccagcggctcgaacaactgctacactggcaacacttgggatgctactctctgccctgacgacgtgacttgcgctgccaactgcgccctggacggcgctgactactcgggcacctacggtgtcaccaccagcggcaactctctgcgcctgaacttcgtcacccaggcgtcgcagaagaacgtcggctctcgtctctatctgatggagaatgacacaacctaccagatcttcaagttgctgaaccaggagttcacctttgacgttgatgtctccaaccttccctgcggtctcaacggtgctctctacctggttgccatggatgccgacggcggcatggccaagtacccaaccaacaaggctggtgcgaagtacggaaccggttactgcgactcccagtgccctcgcgacctgaagttcatcaacggtgaggccaatgttgagggatggcagccttcttccaatgaccccaactctggcattggcaaccacggctcttgctgtgctgagatggacatctgggaggccaacagcatctccaatgcagtcactcctcacccttgcgacaccccgggacaggtcatgtgcaccggcaacaactgtggtggcacttacagcactactcgctatgctggcacttgcgatcctgatggctgcgacttcaacccctaccgcatgggcaaccactccttctacggccccaaacagatcgtcgacaccagctccaagttcactgttgttactcagttcctcaccgatgatggcacctccaccggcaccctcagcgagatcaggcgcttctacgttcagaacggccaggtcatccccaactccgtgtccacgatcagcggcgtctccggcaactccatcaccaccgagttctgcacggcccagaagcaggctttcggcgacactgatgacttcagcaagcacggcggtctgtctggcatgtccgccgccctctcccagggtatggttctcgtcatgagcttgtgggacgaccacgccgccaacatgctctggcttgacagcacctacccgaccaacgccacctcttccacccccggtgccgcccgtggtacttgcgacatctcctccggtgtccccgccgatgttgagtccaacgaccccaacgcctacgtcgtctactccaacatcaaggtcggcccgatcggctctaccttcagcagctctggctctggctctagctccagctccagcaccaccaccaccaccaccgcttccccaaccacgaccacctccagcgcttccagcaccggcactggcgttgctcagcactggggtcagtgcggtggccagggatggaccggtccgaccacctgcgttagcccctacacctgccaggagctgaacccctactactaccagtgcctgtaa

SEQ ID NO: 42 - protein, 532 aa, Talaromyces leycettanus
MASLFSFKMYKAALVLSSLLAATQAQQAGTLTTETHPSLTWQQCSAGGSCTTQNGKVVIDANWRWVHSTSGSNNCYTGNTWDATLCPDDVTCAANCALDGADYSGTYGVTTSGNSLRLNFVTQASQKNVGSRLYLMENDTTYQIFKLLNQEFTFDVDVSNLPCGLNGALYLVAMDADGGMAKYPTNKAGAKYGTGYCDSQCPRDLKFINGEANVEGWQPSSNDPNSGIGNHGSCCAEMDIWEANSISNAVTPHPCDTPGQVMCTGNNCGGTYSTTRYAGTCDPDGCDFNPYRMGNHSFYGPKQIVDTSSKFTVVTQFLTDDGTSTGTLSEIRRFYVQNGQVIPNSVSTISGVSGNSITTEFCTAQKQAFGDTDDFSKHGGLSGMSAALSQGMVLVMSLWDDHAANMLWLDSTYPTNATSSTPGAARGTCDISSGVPADVESNDPNAYVVYSNIKVGPIGSTFSSSGSGSSSSSSTTTTTTASPTTTTSSASSTGTGVAQHWGQCGGQGWTGPTTCVSPYTCQELNPYYYQCL

SEQ ID NO: 43 - DNA, 1599 bp, Talaromyces leycettanus
  sig_peptide (1)..(25)
  CDS (1)..(1596)
  mat_peptide (76)..(1596)
atggcgtcctctctctcttacaggatctacaagaatgctctcatcttctcttctctcctggccgctgcccagggtcagcagattggtacctaccagacggagacccatccgcctctgacctggcagacatgcaccagcggcggcagttgcacgaccaaccaaggctccatcgtcctcgatgccaactggcgctgggtgcacgaggtcggcagcaccaccaactgctacaccggcaatacctgggacacctccatctgcagcacggatacgacctgcgctcagcaatgtgccgtcgatggtgccgactacgagggcacctatggtatcacgaccagcggcagccaggtccgcatcaacttcgtcaccaacaactcgaacggaaagaacgtcggcgcgcgtgtctacatgatggcggacaacacccactaccaaatttaccagctgctgaaccaggagttcacctttgatgtcgacgtgtccaacctgccttgcggcctcaacggtgccctctactttgtggtcatggacgccgatggtggtgtctccaagtatcccaacaacaaggctggtgcccagtacggtgtcggttactgcgactcccagtgtcccagagacctcaaattcatccagggacaggccaacgtcgagggctggcaaccgtcgtccaacaacgccaataccggcctgggcaaccacggctcctgctgtgctgaactggacgtctgggagtcgaacagcatctcccaggccctcactccccacccctgcgacactcccaccaataccctgtgcaccggtgatagctgcggtggcacatacagcagcaaccgttatgcgggcacttgcgatcctgacggctgcgatttcaacccctaccgcttgggcaacaccaccttctacggtcctggcaagactattgacaccaccaaacccttcacggttgtgacgcagttcatcacggatgacggcacttccagcggcaccctgtccgaaattaggcgtttctatgtccagaacggtgttacgtacgcccagcccaactctgacgtcagcggtatcagcggcaatgccatcaacagtgcttactgcactgcggagaacaccgtcttcaacggtgccggcaccttcgcgcagcacggcggcctggctggcatgagccaggccatgtccaccggtatggtcttggtgatgagcctgtgggatgattactatgccgacatgctctggctcgacagcacctacccaaccaacgacaccgcaagcacgcccggtgcggtccgtggaacctgctctacgtcgtccggtgtccccagccaggtcgaatccgccagcccgaacgcctacgtgacctactcgaacatcaaggttggtcccattggctcgactttcaactctggcggctctggctctggcagcagctccagcactaccacgaccactcacgccagcaccacgacgacgtcctccgcctcgtctacgggaactggcgtggcccaacactggggccagtgtggtggacagggctggaccggcccaacaacctgcgtttccccgtacacttgccaggagctgaacccgtactactaccagtgtctgtag

SEQ ID NO: 44 - protein, 532 aa, Talaromyces leycettanus
MASSLSYRIYKNALIFSSLLAAAQGQQIGTYQTETHPPLTWQTCTSGGSCTTNQGSIVLDANWRWVHEVGSTTNCYTGNTWDTSICSTDTTCAQQCAVDGADYEGTYGITTSGSQVRINFVTNNSNGKNVGARVYMMADNTHYQIYQLLNQEFTFDVDVSNLPCGLNGALYFVVMDADGGVSKYPNNKAGAQYGVGYCDSQCPRDLKFIQGQANVEGWQPSSNNANTGLGNHGSCCAELDVWESNSISQALTPHPCDTPTNTLCTGDSCGGTYSSNRYAGTCDPDGCDFNPYRLGNTTFYGPGKTIDTTKPFTVVTQFITDDGTSSGTLSEIRRFYVQNGVTYAQPNSDVSGISGNAINSAYCTAENTVFNGAGTFAQHGGLAGMSQAMSTGMVLVMSLWDDYYADMLWLDSTYPTNDTASTPGAVRGTCSTSSGVPSQVESASPNAYVTYSNIKVGPIGSTFNSGGSGSGSSSSTTTTTHASTTTTSSASSTGTGVAQHWGQCGGQGWTGPTTCVSPYTCQELNPYYYQCL

SEQ ID NO: 45 - DNA, 1507 bp, Talaromyces byssochlamydoides
  exon (1)..(603)
  CDS (1)..(603)
  sig_peptide (1)..(18)
  mat_peptide (55)..(1504)
  Intron (604)..(667)
  exon (668)..(1235)
  CDS (668)..(1235)
  Intron (1236)..(1310)
  exon (1311)..(1504)
  CDS (1311)..(1504)
atgtttcgacgggctcttttcctgtcctcttccgccttccttgctgtcaaagcccagcagatcggcacggtcagtccggagaaccatccgcccctggcatgggagcagtgcactgcccctgggagttgcacgactgtgaatggtgcggtcgtccttgatgcgaactggcgttgggtccacaatgttgggggatacaccaactgctacactggcaatacctgggacaccacgtactgccctgacgacgtgacctgcgcagagaattgtgcgctggatggcgcagattacgagggcacctacggcgtgaccacctcgggcagctccctgaagctcgatttcgtcaccgggtctaacgtcggatctcgtctctacctgttggagaatgattcgacctatcagatcttcaagcttctgaaccaggaattcacctttgacgtcgacgtttccaatcttccgtgcggattaaacggcgctctgtaccttgttaccatggctgctgacggcggggtgtctcagtacccgaataacaaggccggcgcagcgtatggaaccggttattgcgattcccagtgtccaagggacttgaagtttatcgatggccaggtatgtagagctgtaatcacccatgttgtgaaatcactctcctactgacatggtcgatttataggccaacgttgagggctggcagccgtcttcgaacaacgccaatacaggtattggcaaccatggctcctgctgtgcggagatggatatctgggaagccaacagcatctccaatgcggtgactccgcacccatgcgacacacccggccagacaatgtgcgaggggaacgactgtggtggcacgtattccaccaatcgctatgcaggcacctgcgatcctgacggctgcgacttcaacccctaccgcatgggcaaccattctttctacggccctggggagattgtcgatactacccagcccttcactgtcgtgacacagttccttaccgatgatggcacggatactggcactctcagcgagatcaaacgcttctacgtccaaaacgggaaagtcattcctcagccgaactccgacattgccggcgtgactggcaactcgatcaccagcgagttttgcgatgcccagaagacggctttcggcgacattaacaactttgatacacacggcggtctggccagtatgggagctgcgctgcagcagggtatggttctggtgatgagtctgtgggacggtaggtccttgggagacacccggacgttctatatcaaccagaactgccagaactgacgaattaaaacacttttagattacgcggcaaacatgctgtggttggacagcatttatccaacaaatgcatctgctagcactcctggtgctgctcgtggaacctgttcgacgagctccggtgtcccatcgcaagtcgagtcgcagagccccaacgcctacgtgacgtactccaacattaaagttggaccaatcaactcgaccttcaccacttcgtaa

SEQ ID NO: 46 - protein, 455 aa, Talaromyces byssochlamydoides
MFRRALFLSSSAFLAVKAQQIGTVSPENHPPLAWEQCTAPGSCTTVNGAVVLDANWRWVHNVGGYTNCYTGNTWDTTYCPDDVTCAENCALDGADYEGTYGVTTSGSSLKLDFVTGSNVGSRLYLLENDSTYQIFKLLNQEFTFDVDVSNLPCGLNGALYLVTMAADGGVSQYPNNKAGAAYGTGYCDSQCPRDLKFIDGQANVEGWQPSSNNANTGIGNHGSCCAEMDIWEANSISNAVTPHPCDTPGQTMCEGNDCGGTYSTNRYAGTCDPDGCDFNPYRMGNHSFYGPGEIVDTTQPFTVVTQFLTDDGTDTGTLSEIKRFYVQNGKVIPQPNSDIAGVTGNSITSEFCDAQKTAFGDINNFDTHGGLASMGAALQQGMVLVMSLWDDYAANMLWLDSIYPTNASASTPGAARGTCSTSSGVPSQVESQSPNAYVTYSNIKVGPINSTFTTS

SEQ ID NO: 47 - DNA, 1353 bp, Myceliophthora thermophila
  sig_peptide (1)..(20)
  CDS (1)..(1350)
  mat_peptide (61)..(1350)
atgaagcagtacctccagtacctcgcggcgaccctgcccctggtgggcctggccacggcccagcaggcgggtaacctgcagaccgagactcaccccaggctcacttggtccaagtgcacggccccgggatcctgccaacaggtcaacggcgaggtcgtcatcgactccaactggcgctgggtgcacgacgagaacgcgcagaactgctacgacggcaaccagtggaccaacgcttgcagctctgccaccgactgcgccgagaattgcgcgctcgagggtgccgactaccagggcacctatggcgcctcgaccagcggcaatgccctgacgctcaccttcgtcactaagcacgagtacggcaccaacattggctcgcgcctctacctcatgaacggcgcgaacaagtaccagatgttcaccctcaagggcaacgagctggccttcgacgtcgacctctcggccgtcgagtgcggcctcaacagcgccctctacttcgtggccatggaggaggatggcggtgtgtcgagctacccgaccaacacggccggtgctaagttcggcactgggtactgcgacgcccaatgcgcacgcgacctcaagttcgtcggcggcaagggcaacatcgagggctggaagccgtccaccaacgatgccaatgccggtgtcggtccttatggcgggtgctgcgctgagatcgacgtctgggagtcgaacaagtatgctttcgctttcaccccgcacggttgcgagaaccctaaataccacgtctgcgagaccaccaactgcggtggcacctactccgaggaccgcttcgctggtgactgcgatgccaacggctgcgactacaacccctaccgcatgggcaaccaggacttctacggtcccggcttgacggtcgataccagcaagaagttcaccgtcgtcagccagttcgaggagaacaagctcacccagttcttcgtccaggacggcaagaagattgagatccccggccccaaggtcgagggcatcgatgcggacagcgccgctatcacccctgagctgtgcagtgccctgttcaaggccttcgatgaccgtgaccgcttctcggaggttggcggcttcgatgccatcaacacggccctcagcactcccatggtcctcgtcatgtccatctgggatgatcactacgccaatatgctctggctcgactcgagctacccccctgagaaggctggccagcctggcggtgaccgtggcccgtgtcctcaggactctggcgtcccggccgacgttgaggctcagtaccctaatgccaaggtcatctggtccaacatccgcttcggccccatcggctcgactgtcaacgtctaa

SEQ ID NO: 48 - protein, 450 aa, Myceliophthora thermophila
MKQYLQYLAATLPLVGLATAQQAGNLQTETHPRLTWSKCTAPGSCQQVNGEVVIDSNWRWVHDENAQNCYDGNQWTNACSSATDCAENCALEGADYQGTYGASTSGNALTLTFVTKHEYGTNIGSRLYLMNGANKYQMFTLKGNELAFDVDLSAVECGLNSALYFVAMEEDGGVSSYPTNTAGAKFGTGYCDAQCARDLKFVGGKGNIEGWKPSTNDANAGVGPYGGCCAEIDVWESNKYAFAFTPHGCENPKYHVCETTNCGGTYSEDRFAGDCDANGCDYNPYRMGNQDFYGPGLTVDTSKKFTVVSQFEENKLTQFFVQDGKKIEIPGPKVEGIDADSAAITPELCSALFKAFDDRDRFSEVGGFDAINTALSTPMVLVMSIWDDHYANMLWLDSSYPPEKAGQPGGDRGPCPQDSGVPADVEAQYPNAKVIWSNIRFGPIGSTVNV

SEQ ID NO: 49 - DNA, 1590 bp, Chaetomium thermophilum
  sig_peptide (1)..(18)
  CDS (1)..(1587)
  mat_peptide (55)..(1587)
atgatgtacaagaagttcgccgctctcgccgccctcgtggctggcgccgccgcccagcaggcttgctccctcaccactgagacccaccccagactcacttggaagcgctgcacctctggcggcaactgctcgaccgtgaacggcgccgtcaccatcgatgccaactggcgctggactcacaccgtttccggctcgaccaactgctacaccggcaacgagtgggatacctccatctgctctgatggcaagagctgcgcccagacctgctgcgtcgacggcgctgactactcttcgacctatggtatcaccaccagcggtgactccctgaacctcaagttcgtcaccaagcaccagtacggcaccaatgtcggctctcgtgtctacctgatggagaacgacaccaagtaccagatgttcgagctcctcggcaacgagttcaccttcgatgtcgatgtctctaacctgggctgcggtctcaacggtgccctctacttcgtctccatggacgctgatggtggtatgagcaagtactctggcaacaaggctggcgccaagtacggtaccggctactgcgatgctcagtgcccgcgcgaccttaagttcatcaacggcgaggccaacattgagaactggaccccttcgaccaatgatgccaacgccggtttcggccgctatggcagctgctgctctgagatggatatctgggaggccaacaacatggctactgccttcactcctcacccttgcaccattatcggccagagccgctgcgagggcaacagctgcggtggcacctacagctctgagcgctatgctggtgtttgcgatcctgatggctgcgacttcaacgcctaccgccagggcgacaagaccttctacggcaagggcatgaccgtcgacaccaccaagaagatgaccgtcgtcacccagttccacaagaactcggctggcgtcctcagcgagatcaagcgcttctacgttcaggacggcaagatcattgccaacgccgagtccaagatccccggcaaccccggcaactccatcacccaggagtggtgcgatgcccagaaggtcgccttcggtgacatcgatgacttcaaccgcaagggcggtatggctcagatgagcaaggccctcgagggccctatggtcctggtcatgtccgtctgggatgaccactacgccaacatgctctggctcgactcgacctaccccatcgacaaggccggcacccccggcgccgagcgcggtgcttgcccgaccacctccggtgtccctgccgagattgaggcccaggtccccaacagcaacgtcatcttctccaacatccgcttcggccccatcggctcgaccgtccctggcctcgacggcagcactcccagcaacccgaccgccaccgttgctcctcccacttctaccaccagcgtgagaagcagcactactcagatttccaccccgactagccagcccggcggctgcaccacccagaagtggggccagtgcggtggtatcggctacaccggctgcactaactgcgttgctggcactacctgcactgagctcaacccctggtacagccagtgcctgtaa

SEQ ID NO: 50 - protein, 529 aa, Chaetomium thermophilum
MMYKKFAALAALVAGAAAQQACSLTTETHPRLTWKRCTSGGNCSTVNGAVTIDANWRWTHTVSGSTNCYTGNEWDTSICSDGKSCAQTCCVDGADYSSTYGITTSGDSLNLKFVTKHQYGTNVGSRVYLMENDTKYQMFELLGNEFTFDVDVSNLGCGLNGALYFVSMDADGGMSKYSGNKAGAKYGTGYCDAQCPRDLKFINGEANIENWTPSTNDANAGFGRYGSCCSEMDIWEANNMATAFTPHPCTIIGQSRCEGNSCGGTYSSERYAGVCDPDGCDFNAYRQGDKTFYGKGMTVDTTKKMTVVTQFHKNSAGVLSEIKRFYVQDGKIIANAESKIPGNPGNSITQEWCDAQKVAFGDIDDFNRKGGMAQMSKALEGPMVLVMSVWDDHYANMLWLDSTYPIDKAGTPGAERGACPTTSGVPAEIEAQVPNSNVIFSNIRFGPIGSTVPGLDGSTPSNPTATVAPPTSTTSVRSSTTQISTPTSQPGGCTTQKWGQCGGIGYTGCTNCVAGTTCTELNPWYSQCL

SEQ ID NO: 51 - DNA, 21 bp, Artificial Sequence
  Artificial DNA Primer
cccttgtcgatgcgatgtatc

SEQ ID NO: 52 - DNA, 21 bp, Artificial Sequence
  Artificial DNA Primer
atcctcaattccgtcggtcga

SEQ ID NO: 53 - DNA, 1570 bp, Rasamsonia emersonii
gaatcgatgctcaattcgggatggagatgtcgatcagatggagtataaaagggcagggtgaatccagggtccaggccatctgccatcactcagactcaaacactccatcagcagcttcgaaagcggtctttttgctatcatcatgcttcgacgggctcttcttctatcctcttccgccatccttgctgtcaaggcacagcaggccggcacggcgacggcagagaaccacccgcccctgacatggcaggaatgcaccgcccctgggagctgcaccacccagaacggggcggtcgttcttgatgcgaactggcgttgggtgcacgatgtgaacggatacaccaactgctacacgggcaatacctggaaccccacgtactgccctgacgacgaaacctgcgcccagaactgtgcgctggacggcgcggattacgagggcacctacggcgtgacttcgtcgggcagctccttgaagctcaatttcgtcaccgggtcgaacgtcggatcccgtctctacctgctgcaggacgactcgacctatcagatcttcaagcttctgaaccgcgagtttacctttgacgtcgatgtctccaatcttccgtgcggattgaacggcgctctgtactttgtcgccatggacgccgacggcggcgtgtccaagtacccgaacaacaaggctggtgccaagtacggaaccgggtattgcgactcccaatgcccacgggacctcaagttcatcgacggcgaggtatgtccagtggtaaaatcgatcgtctcgtgaacttctgctgacaggttcgatctacaggccaacgtcgagggctggcagccgtcttcgaacaacgccaacaccggaattggcgaccatggctcctgctgtgcggagatggatgtctgggaagccaacagcatctccaatgcggtcactccgcacccgtgcgacacgccaggccagacgatgtgctctggcgatgactgcggtggcacatactctaacgatcgctacgcgggaacctgcgatcctgacggctgtgacttcaacccttaccgcatgggcaacacttctttctacgggcctggcaagatcatcgataccaccaagcctttcactgtcgtgacgcagttcctcactgatgatggtacggatactggaactctcagcgagatcaagcgcttctacgtccagaacggcaacgtcattccgcagcccaactcggacatcagtggcgtgaccggcaactcgatcacgacggagttctgtactgctcagaagcaggcctttggcgacacggacgacttctctcagcacggtggcctggccaagatgggagcggccatgcagcagggtatggtcctggtgatgagtttgtgggacgactacgccgcgcagatgctgtggctggattccgactacccgacggatgcggaccccacgacccctggtattgcccgtggaacgtgtccgacggactcgggcgtcccatcggatgtcgagtcgcagagccccaactcctacgtgacctactcgaacatcaagtttggtccgatcaactcgaccttcaccgcttcgtga

SEQ ID NO: 54 - DNA, 1368 bp, Rasamsonia emersonii
atgttgcgaagggccttgttgctctcgtcctccgcaatcttggcggtcaaggcacagcaggcaggcaccgcaaccgcagagaaccatcctccgctcacttggcaggaatgtacagcacctggctcctgtacaacccagaacggagcggtcgtgctcgatgcgaactggcgctgggtgcacgatgtcaacggatacacaaactgttatacaggtaacacgtggaaccctacgtattgtcccgacgacgaaacgtgtgcccagaactgtgcgttggatggagcagactacgagggaacgtatggcgtgacctcgtccggctcctccttgaagctcaacttcgtcacgggctcgaacgtcggctcccgcttgtacctcctccaggacgactcgacctaccagatcttcaagctcctcaacagggagttcaccttcgacgtcgatgtctccaacttgccctgtggtctcaacggagccttgtacttcgtcgcgatggatgcagacggaggtgtctcgaagtaccccaacaacaaggcaggtgccaagtatggtactggctactgtgattcgcagtgtcctcgcgatctcaagttcattgacggtgaggcgaacgtggaaggatggcagccctcgtccaacaacgcgaacactggcatcggtgatcacggttcgtgttgtgccgagatggacgtctgggaagccaactccatctcgaacgcggtcacaccgcacccgtgtgatactcctggccagactatgtgttccggagatgattgtggaggcacctattcgaacgaccggtatgcaggcacgtgtgacccggatggctgtgacttcaacccgtaccgcatgggcaacacctccttctatggaccgggtaagatcatcgatacaactaagcccttcaccgtcgtcacgcagttcctcacagatgacggcacggacacaggtactttgtcggagatcaaacgcttctacgtccagaacggaaacgtcatcccccagccgaactccgacatttcgggagtcacaggcaactcgattacgaccgagttctgtacagcccagaaacaggcattcggtgacacggatgatttctcccagcacggaggattggcgaaaatgggagccgcaatgcagcagggaatggtcctcgtgatgtcgctctgggacgactatgcagcccagatgttgtggctcgactcggactaccccacagacgccgatcccacgacacccggtatcgcacgaggcacttgtccgacagattccggagtcccgtcggacgtcgagtcccagtcccccaactcgtacgtcacctattcgaacatcaaattcggtcccatcaactcgacattcacagcctcgtaa

SEQ ID NO: 55 - DNA, 1560 bp, Rasamsonia emersonii
atgttgcgaagggccttgttgctctcgtcctccgcaatcttggcggtcaaggcacagcaggcaggcaccgcaaccgcagagaaccatcctccgctcacttggcaggaatgtacagcacctggctcctgtacaacccagaacggagcggtcgtgctcgatgcgaactggcgctgggtgcacgatgtcaacggatacacaaactgttatacaggtaacacgtggaaccctacgtattgtcccgacgacgaaacgtgtgcccagaactgtgcgttggatggagcagactacgagggaacgtatggcgtgacctcgtccggctcctccttgaagctcaacttcgtcacgggctcgaacgtcggctcccgcttgtacctcctccaggacgactcgacctaccagatcttcaagctcctcaacagggagttcaccttcgacgtcgatgtctccaacttgccctgtggtctcaacggagccttgtacttcgtcgcgatggatgcagacggaggtgtctcgaagtaccccaacaacaaggcaggtgccaagtatggtactggctactgtgattcgcagtgtcctcgcgatctcaagttcattgacggtgaggcgaacgtggaaggatggcagccctcgtccaacaacgcgaacactggcatcggtgatcacggttcgtgttgtgccgagatggacgtctgggaagccaactccatctcgaacgcggtcacaccgcacccgtgtgatactcctggccagactatgtgttccggagatgattgtggaggcacctattcgaacgaccggtatgcaggcacgtgtgacccggatggctgtgacttcaacccgtaccgcatgggcaacacctccttctatggaccgggtaagatcatcgatacaactaagcccttcaccgtcgtcacgcagttcctcacagatgacggcacggacacaggtactttgtcggagatcaaacgcttctacgtccagaacggaaacgtcatcccccagccgaactccgacatttcgggagtcacaggcaactcgattacgaccgagttctgtacagcccagaaacaggcattcggtgacacggatgatttctcccagcacggaggattggcgaaaatgggagccgcaatgcagcagggaatggtcctcgtgatgtcgctctgggacgactatgcagcccagatgttgtggctcgactcggactaccccacagacgccgatcccacgacacccggtatcgcacgaggcacttgtccgacagattccggagtcccgtcggacgtcgagtcccagtcccccaactcgtacgtcacctattcgaacatcaaattcggtcccatcaactcgacattcacagcctcgggtggaaaccctcctggcggaaaccctcctggcacaactacaacacgacggcctgcgactacaacgggttcgtcccctggaccgacccagtcccactacggacagtgtggaggcatcggttattccggtccgaccgtctgtgcgtccggcacaacctgtcaggtcttgaacccttactattcgcagtgtctctaa

SEQ ID NO: 56 - protein, 519 aa, Rasamsonia emersonii
MLRRALLLSSSAILAVKAQQAGTATAENHPPLTWQECTAPGSCTTQNGAVVLDANWRWVHDVNGYTNCYTGNTWNPTYCPDDETCAQNCALDGADYEGTYGVTSSGSSLKLNFVTGSNVGSRLYLLQDDSTYQIFKLLNREFTFDVDVSNLPCGLNGALYFVAMDADGGVSKYPNNKAGAKYGTGYCDSQCPRDLKFIDGEANVEGWQPSSNNANTGIGDHGSCCAEMDVWEANSISNAVTPHPCDTPGQTMCSGDDCGGTYSNDRYAGTCDPDGCDFNPYRMGNTSFYGPGKIIDTTKPFTVVTQFLTDDGTDTGTLSEIKRFYVQNGNVIPQPNSDISGVTGNSITTEFCTAQKQAFGDTDDFSQHGGLAKMGAAMQQGMVLVMSLWDDYAAQMLWLDSDYPTDADPTTPGIARGTCPTDSGVPSDVESQSPNSYVTYSNIKFGPINSTFTASGGNPPGGNPPGTTTTRRPATTTGSSPGPTQSHYGQCGGIGYSGPTVCASGTTCQVLNPYYSQCL

SEQ ID NO: 57 - DNA, 58 bp, Artificial Sequence
  Artificial DNA Primer
ggtcccatcaactcgacattcacagcctcgggtggaaaccctcctggcggaaaccctc

SEQ ID NO: 58 - DNA, 21 bp, Artificial Sequence
  Artificial DNA Primer
atcctcaattccgtcggtcga

SEQ ID NO: 59 - DNA, 28 bp, Artificial Sequence
  Artificial DNA Primer
ccacacttctcttccttcctcaatcctc

SEQ ID NO: 60 - DNA, 1560 bp, Rasamsonia emersonii
atgttgcgaagggccttgttgctctcgtcctccgcaatcttggcggtcaaggcacagcaggcaggcaccgcaaccgcagagaaccatcctccgctcacttggcaggaatgtacagcacctggctcctgtacaacccagaacggagcggtcgtgctcgatgcgaactggcgctgggtgcacgatgtcaacggatacacaaactgttatacaggtaacacgtggaaccctacgtattgtcccgacgacgaaacgtgtgcccagaactgtgcgttggatggagcagactacgagggaacgtatggcgtgacctcgtccggctcctccttgaagctcaacttcgtcacgggctcgaacgtcggctcccgcttgtacctcctccaggacgactcgacctaccagatcttcaagctcctcaacagggagttcaccttcgacgtcgatgtctccaacttgccctgtggtctcaacggagccttgtacttcgtcgcgatggatgcagacggaggtgtctcgaagtaccccaacaacaaggcaggtgccaagtatggtactggctactgtgattcgcagtgtcctcgcgatctcaagttcattgacggtgaggcgaacgtggaaggatggcagccctcgtccaacaacgcgaacactggcatcggtgatcacggttcgtgttgtgccgagatggacgtctgggaagccaactccatctcgaacgcggtcacaccgcacccgtgtgatactcctggccagactatgtgttccggagatgattgtggaggcacctattcgaacgaccggtatgcaggcacgtgtgacccggatggctgtgacttcaacccgtaccgcatgggcaacacctccttctatggaccgggtaagatcatcgatacaactaagcccttcaccgtcgtcacgcagttcctcacagatgacggcacggacacaggtactttgtcggagatcaaacgcttctacgtccagaacggaaacgtcatcccccagccgaactccgacatttcgggagtcacaggcaactcgattacgaccgagttctgtacagcccagaaacaggcattcggtgacacggatgatttctcccagcacggaggattggcgaaaatgggagccgcaatgcagcagggaatggtcctcgtgatgtcgctctgggacgactatgcagcccagatgttgtggctcgactcggactaccccacagacgccgatcccacgacacccggtatcgcacgaggcacttgtccgacagattccggagtcccgtcggacgtcgagtcccagtcccccaactcgtacgtcacctattcgaacatcaaattcggtcccatcaactcgacattcacagcctcgggtggaaaccctcctggcggaaaccctcctggcacaactacaacacgacggcctgcgactacaacgggttcgtcccctggaccgacccagtcccactacggacagtgtggaggcatcggttattccggtccgaccgtctgtgcgtccggcacaacctgtcaggtcttgaacccttactggtcgcagtgtctctaa

SEQ ID NO: 61 - protein, 519 aa, Rasamsonia emersonii
MLRRALLLSSSAILAVKAQQAGTATAENHPPLTWQECTAPGSCTTQNGAVVLDANWRWVHDVNGYTNCYTGNTWNPTYCPDDETCAQNCALDGADYEGTYGVTSSGSSLKLNFVTGSNVGSRLYLLQDDSTYQIFKLLNREFTFDVDVSNLPCGLNGALYFVAMDADGGVSKYPNNKAGAKYGTGYCDSQCPRDLKFIDGEANVEGWQPSSNNANTGIGDHGSCCAEMDVWEANSISNAVTPHPCDTPGQTMCSGDDCGGTYSNDRYAGTCDPDGCDFNPYRMGNTSFYGPGKIIDTTKPFTVVTQFLTDDGTDTGTLSEIKRFYVQNGNVIPQPNSDISGVTGNSITTEFCTAQKQAFGDTDDFSQHGGLAKMGAAMQQGMVLVMSLWDDYAAQMLWLDSDYPTDADPTTPGIARGTCPTDSGVPSDVESQSPNSYVTYSNIKFGPINSTFTASGGNPPGGNPPGTTTTRRPATTTGSSPGPTQSHYGQCGGIGYSGPTVCASGTTCQVLNPYWSQCL

SEQ ID NO: 62 - DNA, 1560 bp, Rasamsonia emersonii
atgttgcgaagggccttgttgctctcgtcctccgcaatcttggcggtcaaggcacagcaggcaggcaccgcaaccgcagagaaccatcctccgctcacttggcaggaatgtacagcacctggctcctgtacaacccagaacggagcggtcgtgctcgatgcgaactggcgctgggtgcacgatgtcaacggatacacaaactgttatacaggtaacacgtggaaccctacgtattgtcccgacgacgaaacgtgtgcccagaactgtgcgttggatggagcagactacgagggaacgtatggcgtgacctcgtccggctcctccttgaagctcaacttcgtcacgggctcgaacgtcggctcccgcttgtacctcctccaggacgactcgacctaccagatcttcaagctcctcaacagggagttcaccttcgacgtcgatgtctccaacttgccctgtggtctcaacggagccttgtacttcgtcgcgatggatgcagacggaggtgtctcgaagtaccccaacaacaaggcaggtgccaagtatggtactggctactgtgattcgcagtgtcctcgcgatctcaagttcattgacggtgaggcgaacgtggaaggatggcagccctcgtccaacaacgcgaacactggcatcggtgatcacggttcgtgttgtgccgagatggacgtctgggaagccaactccatctcgaacgcggtcacaccgcacccgtgtgatactcctggccagactatgtgttccggagatgattgtggaggcacctattcgaacgaccggtatgcaggcacgtgtgacccggatggctgtgacttcaacccgtaccgcatgggcaacacctccttctatggaccgggtaagatcatcgatacaactaagcccttcaccgtcgtcacgcagttcctcacagatgacggcacggacacaggtactttgtcggagatcaaacgcttctacgtccagaacggaaacgtcatcccccagccgaactccgacatttcgggagtcacaggcaactcgattacgaccgagttctgtacagcccagaaacaggcattcggtgacacggatgatttctcccagcacggaggattggcgaaaatgggagccgcaatgcagcagggaatggtcctcgtgatgtcgctctgggacgactatgcagcccagatgttgtggctcgactcggactaccccacagacgccgatcccacgacacccggtatcgcacgaggcacttgtccgacagattccggagtcccgtcggacgtcgagtcccagtcccccaactcgtacgtcacctattcgaacatcaaattcggtcccatcaactcgacattcacagcctcgggtggaaaccctcctggcggaaaccctcctggcacaactacaacacgacggcctgcgactacaacgggttcgtcccctggaccgacccagtcccactggggacagtgtggaggcatcggttattccggtccgaccgtctgtgcgtccggcacaacctgtcaggtcttgaacccttactattcgcagtgtctctaa

SEQ ID NO: 63 - protein, 519 aa, Rasamsonia emersonii
MLRRALLLSSSAILAVKAQQAGTATAENHPPLTWQECTAPGSCTTQNGAVVLDANWRWVHDVNGYTNCYTGNTWNPTYCPDDETCAQNCALDGADYEGTYGVTSSGSSLKLNFVTGSNVGSRLYLLQDDSTYQIFKLLNREFTFDVDVSNLPCGLNGALYFVAMDADGGVSKYPNNKAGAKYGTGYCDSQCPRDLKFIDGEANVEGWQPSSNNANTGIGDHGSCCAEMDVWEANSISNAVTPHPCDTPGQTMCSGDDCGGTYSNDRYAGTCDPDGCDFNPYRMGNTSFYGPGKIIDTTKPFTVVTQFLTDDGTDTGTLSEIKRFYVQNGNVIPQPNSDISGVTGNSITTEFCTAQKQAFGDTDDFSQHGGLAKMGAAMQQGMVLVMSLWDDYAAQMLWLDSDYPTDADPTTPGIARGTCPTDSGVPSDVESQSPNSYVTYSNIKFGPINSTFTASGGNPPGGNPPGTTTTRRPATTTGSSPGPTQSHWGQCGGIGYSGPTVCASGTTCQVLNPYYSQCL

SEQ ID NO: 64 - DNA, 41 bp, Artificial Sequence
  Artificial DNA Primer
ctgtcaggtcttgaacccttactggtcgcagtgtctctaag

SEQ ID NO: 65 - DNA, 32 bp, Artificial Sequence
  Artificial DNA Primer
gtaagggttcaagacctgacaggttgtgccgg

SEQ ID NO: 66 - DNA, 43 bp, Artificial Sequence
  Artificial DNA Primer
ctggaccgacccagtcccactggggacagtgtggaggcatcgg

SEQ ID NO: 67 - DNA, 30 bp, Artificial Sequence
  Artificial DNA Primer
gtgggactgggtcggtccaggggacgaacc

SEQ ID NO: 68 - DNA, 28 bp, Artificial Sequence
  Artificial DNA Primer
ccacacttctcttccttcctcaatcctc

SEQ ID NO: 69 - DNA, 22 bp, Artificial Sequence
  Artificial DNA Primer
gtgaggcgaacgtggaaggatg

SEQ ID NO: 70 - DNA, 25 bp, Artificial Sequence
  Artificial DNA Primer
gtacctgtgtccgtgccgtcatctg

SEQ ID NO: 71 - DNA, 21 bp, Artificial Sequence
  Artificial DNA Primer
atcctcaattccgtcggtcga

SEQ ID NO: 72 - DNA, 1560 bp, Rasamsonia emersonii
atgttgcgaagggccttgttgctctcgtcctccgcaatcttggcggtcaaggcacagcaggcaggcaccgcaaccgcagagaaccatcctccgctcacttggcaggaatgtacagcacctggctcctgtacaacccagaacggagcggtcgtgctcgatgcgaactggcgctgggtgcacgatgtcaacggatacacaaactgttatacaggtaacacgtggaaccctacgtattgtcccgacgacgaaacgtgtgcccagaactgtgcgttggatggagcagactacgagggaacgtatggcgtgacctcgtccggctcctccttgaagctcaacttcgtcacgggctcgaacgtcggctcccgcttgtacctcctccaggacgactcgacctaccagatcttcaagctcctcaacagggagttcaccttcgacgtcgatgtctccaacttgccctgtggtctcaacggagccttgtacttcgtcgcgatggatgcagacggaggtgtctcgaagtaccccaacaacaaggcaggtgccaagtatggtactggctactgtgattcgcagtgtcctcgcgatctcaagttcattgacggtgaggcgaacgtggaaggatggcagccctcgtccaacaacgcgaacactggcatcggtgatcacggttcgtgttgtgccgagatggacgtctgggaagccaactccatctcgaacgcggtcacaccgcacccgtgtgatactcctggccagactatgtgttccggagatgattgtggaggcacctattcgaacgaccggtatgcaggcacgtgtgacccggatggctgtgacttcaacccgtaccgcatgggcaacacctccttctatggaccgggtaagatcatcgatacaactaagcccttcaccgtcgtcacgcagttcctcacagatgacggcacggacacaggtactttgtcggagatcaaacgcttctacgtccagaacggaaacgtcatcccccagccgaactccgacatttcgggagtcacaggcaactcgattacgaccgagttctgtacagcccagaaacaggcattcggtgacacggatgatttctcccagcacggaggattggcgaaaatgggagccgcaatgcagcagggaatggtcctcgtgatgtcgctctgggacgactatgcagcccagatgttgtggctcgactcggactaccccacagacgccgatcccacgacacccggtatcgcacgaggcacttgtccgacagattccggagtcccgtcggacgtcgagtcccagtcccccaactcgtacgtcacctattcgaacatcaaattcggtcccatcaactcgacattcacagcctcgggtggaaaccctcctggcggaaaccctcctggcacaactacaacacgacggcctgcgactacaacgggttcgtcccctggaccgacccagtcccactacggacagtgtggaggcatcggttggtccggtccgaccgtctgtgcgtccggcacaacctgtcaggtcttgaacccttactattcgcagtgtctctaa

SEQ ID NO: 73 - protein, 519 aa, Rasamsonia emersonii
MLRRALLLSSSAILAVKAQQAGTATAENHPPLTWQECTAPGSCTTQNGAVVLDANWRWVHDVNGYTNCYTGNTWNPTYCPDDETCAQNCALDGADYEGTYGVTSSGSSLKLNFVTGSNVGSRLYLLQDDSTYQIFKLLNREFTFDVDVSNLPCGLNGALYFVAMDADGGVSKYPNNKAGAKYGTGYCDSQCPRDLKFIDGEANVEGWQPSSNNANTGIGDHGSCCAEMDVWEANSISNAVTPHPCDTPGQTMCSGDDCGGTYSNDRYAGTCDPDGCDFNPYRMGNTSFYGPGKIIDTTKPFTVVTQFLTDDGTDTGTLSEIKRFYVQNGNVIPQPNSDISGVTGNSITTEFCTAQKQAFGDTDDFSQHGGLAKMGAAMQQGMVLVMSLWDDYAAQMLWLDSDYPTDADPTTPGIARGTCPTDSGVPSDVESQSPNSYVTYSNIKFGPINSTFTASGGNPPGGNPPGTTTTRRPATTTGSSPGPTQSHYGQCGGIGWSGPTVCASGTTCQVLNPYYSQCL

SEQ ID NO: 74 - DNA, 44 bp, Artificial Sequence
  Artificial DNA Primer
ggacagtgtggaggcatcggttggtccggtccgaccgtctgtgc

SEQ ID NO: 75 - DNA, 32 bp, Artificial Sequence
  Artificial DNA Primer
accgatgcctccacactgtccgtagtgggact

SEQ ID NO: 76 - DNA, 1599 bp, Aspergillus fumigatus
atgctggcctccaccttctcctaccgcatgtacaagaccgcgctcatcctggccgcccttctgggctctggccaggctcagcaggtcggtacttcccaggcggaagtgcatccgtccatgacctggcagagctgcacggctggcggcagctgcaccaccaacaacggcaaggtggtcatcgacgcgaactggcgttgggtgcacaaagtcggcgactacaccaactgctacaccggcaacacctgggacacgactatctgccctgacgatgcgacctgcgcatccaactgcgcccttgagggtgccaactacgaatccacctatggtgtgaccgccagcggcaattccctccgcctcaacttcgtcaccaccagccagcagaagaacattggctcgcgtctgtacatgatgaaggacgactcgacctacgagatgtttaagctgctgaaccaggagttcaccttcgatgtcgatgtctccaacctcccctgcggtctcaacggtgctctgtactttgtcgccatggacgccgacggtggcatgtccaagtacccaaccaacaaggccggtgccaagtacggtactggatactgtgactcgcagtgccctcgcgacctcaagttcatcaacggtcaggccaacgttgaagggtggcagccctcctccaacgatgccaatgcgggtaccggcaaccacgggtcctgctgcgcggagatggatatctgggaggccaacagcatctccacggccttcaccccccatccgtgcgacacgcccggccaggtgatgtgcaccggtgatgcctgcggtggcacctacagctccgaccgctacggcggcacctgcgaccccgacggatgtgatttcaactccttccgccagggcaacaagaccttctacggccctggcatgaccgtcgacaccaagagcaagtttaccgtcgtcacccagttcatcaccgacgacggcacctccagcggcaccctcaaggagatcaagcgcttctacgtgcagaacggcaaggtgatccccaactcggagtcgacctggaccggcgtcagcggcaactccatcaccaccgagtactgcaccgcccagaaaagcctgttccaggaccagaacgtcttcgaaaagcacggcggcctcgagggcatgggtgctgccctcgcccagggcatggttctcgtcatgtccctgtgggatgatcactcggccaacatgctctggctcgacagcaactacccgaccactgcctcttccaccactcccggcgtcgcccgtggtacctgcgacatctcctccggcgtccctgcggatgtcgaggcgaaccaccccgacgcctacgtcgtctactccaacatcaaggtcggccccatcggctcgaccttcaacagcggtggctcgaaccccggtggcggaaccaccacgacaactaccacccagcctactaccaccacgaccacggctggaaaccctggcggcaccggagtcgcacagcactatggccagtgtggtggaatcggatggaccggacccacaacctgtgccagcccttatacctgccagaagctgaatgattattactctcagtgcctgtag

SEQ ID NO: 77 - DNA, 1599 bp, Aspergillus fumigatus; identical to SEQ ID NO: 76

SEQ ID NO: 78 - protein, 532 aa, Aspergillus fumigatus; identical to SEQ ID NO: 36

SEQ ID NO: 79 - DNA, 1599 bp, Aspergillus fumigatus
atgttggcctccacgttctcctatcgcatgtacaaaacagcgctcatcttggcagccctcttgggctcgggacaggcacagcaggtcggaacctcgcaggccgaggtccatccttccatgacgtggcagtcgtgtacagcgggtggttcgtgtaccacaaacaacggtaaagtcgtgatcgatgcaaactggaggtgggtgcacaaggtcggcgactacaccaactgttacacaggcaacacatgggatacaaccatctgtcccgacgatgccacttgtgcatccaactgtgcactcgagggtgccaactatgagtcgacgtacggagtgaccgcctccggaaactcgctcaggctcaacttcgtcacaacttcccagcagaagaacatcggctcgcggttgtatatgatgaaagacgattccacttacgagatgttcaagctcctcaaccaggaattcactttcgatgtcgacgtctccaacctcccttgtggcttgaacggagcgctctacttcgtcgccatggatgcggatggaggcatgtccaagtatcctaccaacaaagcaggagccaagtatggtacaggttactgtgattcccagtgtcccagggatctcaagttcatcaacggtcaggccaacgtcgagggttggcagccttcgtcgaacgatgccaacgcaggtaccggcaaccacggttcctgttgtgccgaaatggacatttgggaagcgaactcgatctcgacggcgttcactcctcacccgtgtgatacacccggacaggtgatgtgtacaggcgacgcctgtggcggaacctactcgtcggatcgatatggcggtacgtgtgaccccgacggctgtgacttcaactccttcaggcagggcaacaaaacattctatggacctggcatgacggtggatacaaagtcgaaattcacagtcgtcactcagttcatcaccgacgatggtacgtcctcgggtaccttgaaggagatcaaaaggttctatgtccagaacggaaaggtcatcccgaactcggagtccacgtggacaggagtgtcgggtaactccatcactacggagtattgtacagcccagaagtcgctcttccaggatcagaacgtcttcgagaaacatggaggcttggaaggaatgggtgccgcattggcccagggtatggtcctcgtcatgtccttgtgggacgaccactcggccaacatgctctggttggattccaactaccccaccactgcctcgtccacgacaccgggtgtcgcacgcggaacttgtgatatctcctcgggagtgcctgcagacgtcgaggcgaaccatcccgacgcctacgtggtctactcgaacattaaggtgggacccatcggttcgacattcaactccggaggctcgaaccctggaggcggaacgaccactactacaacgactcagccgacaacaacaactaccacagcaggcaaccctggaggtacaggtgtggcccagcactacggacagtgtggcggtatcggatggacaggacctactacttgtgcatcgccttatacctgtcagaaattgaacgactactactcgcagtgtttgtaa

SEQ ID NO: 80 - DNA, 25 bp, Artificial Sequence
  Artificial DNA Primer
gtgatacacccggacaggtgatgtg

SEQ ID NO: 81 - DNA, 25 bp, Artificial Sequence
  Artificial DNA Primer
ccatatcgatccgacgagtaggttc

SEQ ID NO: 82 - DNA, 1507 bp, Talaromyces byssochlamydoides; identical to SEQ ID NO: 45

SEQ ID NO: 83 - protein, 455 aa, Talaromyces byssochlamydoides; identical to SEQ ID NO: 46

SEQ ID NO: 84 - DNA, 1705 bp, Talaromyces byssochlamydoides
atgtttcgacgggctcttttcctgtcctcttccgccttccttgctgtcaaagcccagcagatcggcacggtcagtccggagaaccatccgcccctggcatgggagcagtgcactgcccctgggagttgcacgactgtgaatggtgcggtcgtccttgatgcgaactggcgttgggtccacaatgttgggggatacaccaactgctacactggcaatacctgggacaccacgtactgccctgacgacgtgacctgcgcagagaattgtgcgctggatggcgcagattacgagggcacctacggcgtgaccacctcgggcagctccctgaagctcgatttcgtcaccgggtctaacgtcggatctcgtctctacctgttggagaatgattcgacctatcagatcttcaagcttctgaaccaggaattcacctttgacgtcgacgtttccaatcttccgtgcggattaaacggcgctctgtaccttgttaccatggctgctgacggcggggtgtctcagtacccgaataacaaggccggcgcagcgtatggaaccggttattgcgattcccagtgtccaagggacttgaagtttatcgatggccaggtatgtagagctgtaatcacccatgttgtgaaatcactctcctactgacatggtcgatttataggccaacgttgagggctggcagccgtcttcgaacaacgccaatacaggtattggcaaccatggctcctgctgtgcggagatggatatctgggaagccaacagcatctccaatgcggtgactccgcacccatgcgacacacccggccagacaatgtgcgaggggaacgactgtggtggcacgtattccaccaatcgctatgcaggcacctgcgatcctgacggctgcgacttcaacccctaccgcatgggcaaccattctttctacggccctggggagattgtcgatactacccagcccttcactgtcgtgacacagttccttaccgatgatggcacggatactggcactctcagcgagatcaaacgcttctacgtccaaaacgggaaagtcattcctcagccgaactccgacattgccggcgtgactggcaactcgatcaccagcgagttttgcgatgcccagaagacggctttcggcgacattaacaactttgatacacacggcggtctggccagtatgggagctgcgctgcagcagggtatggttctggtgatgagtctgtgggacggtaggtccttgggagacacccggacgttctatatcaaccagaactgccagaactgacgaattaaaacacttttagattacgcggcaaacatgctgtggttggacagcatttatccaacaaatgcatctgctagcactcctggtgctgctcgtggaacctgttcgacgagctccggtgtcccatcgcaagtcgagtcgcagagccccaacgcctacgtgacgtactccaacattaaagttggaccaatcaactcgaccttcaccacttcgggctcgaaccctggaggcggaacgaccactactacaacgactcagccgacaacaacaactaccacagcaggcaaccctggaggtacaggtgtggcccagcactacggacagtgtggcggtatcggatggacaggacctactacttgtgcatcgccttatacctgtcagaaattgaacgactactactcgcagtgtttgtaa

SEQ ID NO: 85 - protein, 521 aa, Talaromyces byssochlamydoides
MFRRALFLSSSAFLAVKAQQIGTVSPENHPPLAWEQCTAPGSCTTVNGAVVLDANWRWVHNVGGYTNCYTGNTWDTTYCPDDVTCAENCALDGADYEGTYGVTTSGSSLKLDFVTGSNVGSRLYLLENDSTYQIFKLLNQEFTFDVDVSNLPCGLNGALYLVTMAADGGVSQYPNNKAGAAYGTGYCDSQCPRDLKFIDGQANVEGWQPSSNNANTGIGNHGSCCAEMDIWEANSISNAVTPHPCDTPGQTMCEGNDCGGTYSTNRYAGTCDPDGCDFNPYRMGNHSFYGPGEIVDTTQPFTVVTQFLTDDGTDTGTLSEIKRFYVQNGKVIPQPNSDIAGVTGNSITSEFCDAQKTAFGDINNFDTHGGLASMGAALQQGMVLVMSLWDDYAANMLWLDSIYPTNASASTPGAARGTCSTSSGVPSQVESQSPNAYVTYSNIKVGPINSTFTTSGSNPGGGTTTTTTTQPTTTTTTAGNPGGTGVAQHYGQCGGIGWTGPTTCASPYTCQKLNDYYSQCL

SEQ ID NO: 86 - DNA, 50 bp, Artificial Sequence
  Artificial DNA Primer
caatcaactcgaccttcaccacttcgggctcgaaccctggaggcggaacg

SEQ ID NO: 87 - DNA, 34 bp, Artificial Sequence
  Artificial DNA Primer
ctagatctcgagttacaaacactgcgagtagtag

SEQ ID NO: 88 - DNA, 26 bp, Artificial Sequence
  Artificial DNA Primer
cgaagtggtgaaggtcgagttgattg

SEQ ID NO: 89 - DNA, 1599 bp, Aspergillus fumigatus
atgttggcctccacgttctcctatcgcatgtacaaaacagcgctcatcttggcagccctcttgggctcgggacaggcacagcaggtcggaacctcgcaggccgaggtccatccttccatgacgtggcagtcgtgtacagcgggtggttcgtgtaccacaaacaacggtaaagtcgtgatcgatgcaaactggaggtgggtgcacaaggtcggcgactacaccaactgttacacaggcaacacatgggatacaaccatctgtcccgacgatgccacttgtgcatccaactgtgcactcgagggtgccaactatgagtcgacgtacggagtgaccgcctccggaaactcgctcaggctcaacttcgtcacaacttcccagcagaagaacatcggctcgcggttgtatatgatgaaagacgattccacttacgagatgttcaagctcctcaaccaggaattcactttcgatgtcgacgtctccaacctcccttgtggcttgaacggagcgctctacttcgtcgccatggatgcggatggaggcatgtccaagtatcctaccaacaaagcaggagccaagtatggtacaggttactgtgattcccagtgtcccagggatctcaagttcatcaacggtcaggccaacgtcgagggttggcagccttcgtcgaacgatgccaacgcaggtaccggcaaccacggttcctgttgtgccgaaatggacatttgggaagcgaactcgatctcgacggcgttcactcctcacccgtgtgatacacccggacaggtgatgtgtacaggcgacgcctgtggcggaacctactcgtcggatcgatatggcggtacgtgtgaccccgacggctgtgacttcaactccttcaggcagggcaacaaaacattctatggacctggcatgacggtggatacaaagtcgaaattcacagtcgtcactcagttcatcaccgacgatggtacgtcctcgggtaccttgaaggagatcaaaaggttctatgtccagaacggaaaggtcatcccgaactcggagtccacgtggacaggagtgtcgggtaactccatcactacggagtattgtacagcccagaagtcgctcttccaggatcagaacgtcttcgagaaacatggaggcttggaaggaatgggtgccgcattggcccagggtatggtcctcgtcatgtccttgtgggacgaccactcggccaacatgctctggttggattccaactaccccaccactgcctcgtccacgacaccgggtgtcgcacgcggaacttgtgatatctcctcgggagtgcctgcagacgtcgaggcgaaccatcccgacgcctacgtggtctactcgaacattaaggtgggacccatcggttcgacattcaactccggaggctcgaaccctggaggcggaacgaccactactacaacgactcagccgacaacaacaactaccacagcaggcaaccctggaggtacaggtgtggcccagcactggggacagtgtggcggtatcggatggacaggacctactacttgtgcatcgccttatacctgtcagaaattgaacgactactactcgcagtgtttgtaa

SEQ ID NO: 90 - protein, 532 aa, Aspergillus fumigatus
MLASTFSYRMYKTALILAALLGSGQAQQVGTSQAEVHPSMTWQSCTAGGSCTTNNGKVVIDANWRWVHKVGDYTNCYTGNTWDTTICPDDATCASNCALEGANYESTYGVTASGNSLRLNFVTTSQQKNIGSRLYMMKDDSTYEMFKLLNQEFTFDVDVSNLPCGLNGALYFVAMDADGGMSKYPTNKAGAKYGTGYCDSQCPRDLKFINGQANVEGWQPSSNDANAGTGNHGSCCAEMDIWEANSISTAFTPHPCDTPGQVMCTGDACGGTYSSDRYGGTCDPDGCDFNSFRQGNKTFYGPGMTVDTKSKFTVVTQFITDDGTSSGTLKEIKRFYVQNGKVIPNSESTWTGVSGNSITTEYCTAQKSLFQDQNVFEKHGGLEGMGAALAQGMVLVMSLWDDHSANMLWLDSNYPTTASSTTPGVARGTCDISSGVPADVEANHPDAYVVYSNIKVGPIGSTFNSGGSNPGGGTTTTTTTQPTTTTTTAGNPGGTGVAQHWGQCGGIGWTGPTTCASPYTCQKLNDYYSQCL

SEQ ID NO: 91 - DNA, 1599 bp, Aspergillus fumigatus
atgttggcctccacgttctcctatcgcatgtacaaaacagcgctcatcttggcagccctcttgggctcgggacaggcacagcaggtcggaacctcgcaggccgaggtccatccttccatgacgtggcagtcgtgtacagcgggtggttcgtgtaccacaaacaacggtaaagtcgtgatcgatgcaaactggaggtgggtgcacaaggtcggcgactacaccaactgttacacaggcaacacatgggatacaaccatctgtcccgacgatgccacttgtgcatccaactgtgcactcgagggtgccaactatgagtcgacgtacggagtgaccgcctccggaaactcgctcaggctcaacttcgtcacaacttcccagcagaagaacatcggctcgcggttgtatatgatgaaagacgattccacttacgagatgttcaagctcctcaaccaggaattcactttcgatgtcgacgtctccaacctcccttgtggcttgaacggagcgctctacttcgtcgccatggatgcggatggaggcatgtccaagtatcctaccaacaaagcaggagccaagtatggtacaggttactgtgattcccagtgtcccagggatctcaagttcatcaacggtcaggccaacgtcgagggttggcagccttcgtcgaacgatgccaacgcaggtaccggcaaccacggttcctgttgtgccgaaatggacatttgggaagcgaactcgatctcgacggcgttcactcctcacccgtgtgatacacccggacaggtgatgtgtacaggcgacgcctgtggcggaacctactcgtcggatcgatatggcggtacgtgtgaccccgacggctgtgacttcaactccttcaggcagggcaacaaaacattctatggacctggcatgacggtggatacaaagtcgaaattcacagtcgtcactcagttcatcaccgacgatggtacgtcctcgggtaccttgaaggagatcaaaaggttctatgtccagaacggaaaggtcatcccgaactcggagtccacgtggacaggagtgtcgggtaactccatcactacggagtattgtacagcccagaagtcgctcttccaggatcagaacgtcttcgagaaacatggaggcttggaaggaatgggtgccgcattggcccagggtatggtcctcgtcatgtccttgtgggacgaccactcggccaacatgctctggttggattccaactaccccaccactgcctcgtccacgacaccgggtgtcgcacgcggaacttgtgatatctcctcgggagtgcctgcagacgtcgaggcgaaccatcccgacgcctacgtggtctactcgaacattaaggtgggacccatcggttcgacattcaactccggaggctcgaaccctggaggcggaacgaccactactacaacgactcagccgacaacaacaactaccacagcaggcaaccctggaggtacaggtgtggcccagcactacggacagtgtggcggtatcggatggacaggacctactacttgtgcatcgccttatacctgtcagaaattgaacgactggtactcgcagtgtttgtaa

SEQ ID NO: 92 - protein, 532 aa, Aspergillus fumigatus
MLASTFSYRMYKTALILAALLGSGQAQQVGTSQAEVHPSMTWQSCTAGGSCTTNNGKVVIDANWRWVHKVGDYTNCYTGNTWDTTICPDDATCASNCALEGANYESTYGVTASGNSLRLNFVTTSQQKNIGSRLYMMKDDSTYEMFKLLNQEFTFDVDVSNLPCGLNGALYFVAMDADGGMSKYPTNKAGAKYGTGYCDSQCPRDLKFINGQANVEGWQPSSNDANAGTGNHGSCCAEMDIWEANSISTAFTPHPCDTPGQVMCTGDACGGTYSSDRYGGTCDPDGCDFNSFRQGNKTFYGPGMTVDTKSKFTVVTQFITDDGTSSGTLKEIKRFYVQNGKVIPNSESTWTGVSGNSITTEYCTAQKSLFQDQNVFEKHGGLEGMGAALAQGMVLVMSLWDDHSANMLWLDSNYPTTASSTTPGVARGTCDISSGVPADVEANHPDAYVVYSNIKVGPIGSTFNSGGSNPGGGTTTTTTTQPTTTTTTAGNPGGTGVAQHYGQCGGIGWTGPTTCASPYTCQKLNDWYSQCL

SEQ ID NO: 93 - DNA, 1705 bp, Talaromyces byssochlamydoides
atgtttcgacgggctcttttcctgtcctcttccgccttccttgctgtcaaagcccagcagatcggcacggtcagtccggagaaccatccgcccctggcatgggagcagtgcactgcccctgggagttgcacgactgtgaatggtgcggtcgtccttgatgcgaactggcgttgggtccacaatgttgggggatacaccaactgctacactggcaatacctgggacaccacgtactgccctgacgacgtgacctgcgcagagaattgtgcgctggatggcgcagattacgagggcacctacggcgtgaccacctcgggcagctccctgaagctcgatttcgtcaccgggtctaacgtcggatctcgtctctacctgttggagaatgattcgacctatcagatcttcaagcttctgaaccaggaattcacctttgacgtcgacgtttccaatcttccgtgcggattaaacggcgctctgtaccttgttaccatggctgctgacggcggggtgtctcagtacccgaataacaaggccggcgcagcgtatggaaccggttattgcgattcccagtgtccaagggacttgaagtttatcgatggccaggtatgtagagctgtaatcacccatgttgtgaaatcactctcctactgacatggtcgatttataggccaacgttgagggctggcagccgtcttcgaacaacgccaatacaggtattggcaaccatggctcctgctgtgcggagatggatatctgggaagccaacagcatctccaatgcggtgactccgcacccatgcgacacacccggccagacaatgtgcgaggggaacgactgtggtggcacgtattccaccaatcgctatgcaggcacctgcgatcctgacggctgcgacttcaacccctaccgcatgggcaaccattctttctacggccctggggagattgtcgatactacccagcccttcactgtcgtgacacagttccttaccgatgatggcacggatactggcactctcagcgagatcaaacgcttctacgtccaaaacgggaaagtcattcctcagccgaactccgacattgccggcgtgactggcaactcgatcaccagcgagttttgcgatgcccagaagacggctttcggcgacattaacaactttgatacacacggcggtctggccagtatgggagctgcgctgcagcagggtatggttctggtgatgagtctgtgggacggtaggtccttgggagacacccggacgttctatatcaaccagaactgccagaactgacgaattaaaacacttttagattacgcggcaaacatgctgtggttggacagcatttatccaacaaatgcatctgctagcactcctggtgctgctcgtggaacctgttcgacgagctccggtgtcccatcgcaagtcgagtcgcagagccccaacgcctacgtgacgtactccaacattaaagttggaccaatcaactcgaccttcaccacttcgggctcgaaccctggaggcggaacgaccactactacaacgactcagccgacaacaacaactaccacagcaggcaaccctggaggtacaggtgtggcccagcactacggacagtgtggcggtatcggatggacaggacctactacttgtgcatcgccttatacctgtcagaaattgaacgactggtactcgcagtgtttgtaa

SEQ ID NO: 94 - protein, 521 aa, Talaromyces byssochlamydoides
MFRRALFLSSSAFLAVKAQQIGTVSPENHPPLAWEQCTAPGSCTTVNGAVVLDANWRWVHNVGGYTNCYTGNTWDTTYCPDDVTCAENCALDGADYEGTYGVTTSGSSLKLDFVTGSNVGSRLYLLENDSTYQIFKLLNQEFTFDVDVSNLPCGLNGALYLVTMAADGGVSQYPNNKAGAAYGTGYCDSQCPRDLKFIDGQANVEGWQPSSNNANTGIGNHGSCCAEMDIWEANSISNAVTPHPCDTPGQTMCEGNDCGGTYSTNRYAGTCDPDGCDFNPYRMGNHSFYGPGEIVDTTQPFTVVTQFLTDDGTDTGTLSEIKRFYVQNGKVIPQPNSDIAGVTGNSITSEFCDAQKTAFGDINNFDTHGGLASMGAALQQGMVLVMSLWDDYAANMLWLDSIYPTNASASTPGAARGTCSTSSGVPSQVESQSPNAYVTYSNIKVGPINSTFTTSGSNPGGGTTTTTTTQPTTTTTTAGNPGGTGVAQHYGQCGGIGWTGPTTCASPYTCQKLNDWYSQCL

SEQ ID NO: 95 - DNA, 43 bp, Artificial Sequence
  Artificial DNA Primer
gtacaggtgtggcccagcactggggacagtgtggcggtatcgg

SEQ ID NO: 96 - DNA, 31 bp, Artificial Sequence
  Artificial DNA Primer
gtgctgggccacacctgtacctccagggttg

SEQ ID NO: 97 - DNA, 49 bp, Artificial Sequence
  Artificial DNA Primer
atacctgtcagaaattgaacgactggtactcgcagtgtttgtaagcttc

SEQ ID NO: 98 - DNA, 32 bp, Artificial Sequence
  Artificial DNA Primer
gtcgttcaatttctgacaggtataaggcgatg

SEQ ID NO: 99 - DNA, 23 bp, Artificial Sequence
  Artificial DNA Primer
cctcagccgaactccgacattgc

SEQ ID NO: 100 - DNA, 23 bp, Artificial Sequence
  Artificial DNA Primer
gcaatgtcggagttcggctgagg